European Patent Specification EP 4 401 757 B1, published March 25, 2026. Title: GENE EDITING TOOLS. Applicant: LIFE TECHNOLOGIES CORPORATION. Application WO. The sequence listing filed with the application follows.

SEQUENCE LISTING (299 sequences)

SEQ ID NO: 1 - protein, 196 aa, synthetic construct
  REGION 1..196: note = Synthetic Construct
QLVKSELEEKKSELRHKLKYVPHEYIELIEIARNSTQDRILEMKVMEFFMKVYGYRGKHLGGSRKPDGAIYTVGSPIDYGVIVDTKAYSGGYNLPIGQADEMQRYVEENQTRNKHINPNEWWKVYPSSVTEFKFLFVSGHFKGNYKAQLTRLNHITNCNGAVLSVEELLIGGEMIKAGTLTLEEVRRKFNNGEINF

SEQ ID NO: 2 - protein, 200 aa, synthetic construct
  REGION 1..200: note = Synthetic Construct
GEGIKSNISLLKDELRGQISHISHEYLSLIDLAFDSKQNRLFEMKVLELLVNEYGFKGRHLGGSRKPDGIVYSTTLEDNFGIIVDTKAYSEGYSLPISQADEMERYVRENSNRDEEVNPNKWWENFSEEVKKYYFVFISGSFKGKFEEQLRRLSMTTGVNGSAVNVVNLLLGAEKIRSGEMTIEELERAMFNNSEFILKY

SEQ ID NO: 3 - protein, 201 aa, synthetic construct
  REGION 1..201: note = Synthetic Construct
PTARLEGKSEVETIKEQMRGELTHLSHEYLGLLDLAYDSKQNRLFELKTMQLLTEECGFEGLHLGGSRKPDGIVYTKDENEQVGKENYGIIIDTKAYSGGYSLPISQADEMERYIGENQTRDIRINPNEWWKNFGDGVTEYYYLFVAGHFKGKYQEQIDRINCNKNIKGAAVSIQQLLRIVNDYKAGKLTHEDMKLKIFHY

SEQ ID NO: 4 - protein, 200 aa, synthetic construct
  REGION 1..200: note = Synthetic Construct
GVTERLVKGEMEKKKAELRHKLKHVPHEYIELIEIAQDSKQNRLLEFKVVEFFKEVYGYHGKHLGGSRKPDGALYTKGLGADHGIILDTKAYKDGYSLPISQADEMQRYVDENNKRDAIINPNEWWKVYPSSISDFKFLFVSGYFKGDTKKQLTRVSNLTKRKGAVLSVEQLLLGGEKIKDGSITLEDVAAKFNNDEIVF

SEQ ID NO: 5 - protein, 200 aa, synthetic construct
  REGION 1..200: note = Synthetic Construct
GVTEPLVKGEMEKKKSDLRHKLKHVPHEYIELIEIAQDSKQNRLFEFKVVEFLKEGYDYNGKHLGGSRKPDGALYTNGLKTDYGIILDTKAYKDGYSLPISQADEMQRYVDENNNRNAIINPNEWWKVYPNSILDFKFLFVSGFFKGDYKKQLARVSNLTKRKGAVLSVEQLLLGGEKIKDGSLTLEDVGDKFNNDEIIF

SEQ ID NO: 6 - protein, 214 aa, synthetic construct
  REGION 1..214: note = Synthetic Construct
GLLFPEAQSFLPVKSQVSILKDYLRSCLSHVDHKYLILLDLGFDGTSDRDYEIQTAQLLTAELSFLGGRLGDTRKPDVCIYYEDNGLIIDNKAYGKGYSLPIKQADEMYRYIEENKERSELLNPNCWWNIFDEGVKTFRFAFLSGEFTGGFKDRLNHISMRSGIKGAAVNSANLLIIAEQLKSGTMSYEEFFQLFDQNDEITVPHLSLQGGLIL

SEQ ID NO: 7 - protein, 201 aa, synthetic construct
  REGION 1..201: note = Synthetic Construct
MSQSFTKSDFEETKEQIRGKLLHLPHEYLSLIDLAYDSKQNRLFEMKTLGLLTEECGYQGLHLGGSRKPDGIIYTSSEKYNYGVIIDTKAYSRGYNLPISQADEMERYIGENQTRDAKINPNKWWKHFPEEVNEFYFMFVSGHFIGNFKAQIMRISRNKAINGTAIAVANLLLCVEAYKAGQLTHEVIKTKVFNNGEFELL

SEQ ID NO: 8 - protein, 204 aa, synthetic construct
  REGION 1..204: note = Synthetic Construct
VPKKLAKSSQSETKEKLREKLRNLPHEYLSLVDLAYDSKQNRLFEMKVIELLTEECGFQGLHLGGSRRPDGVLYTAGLTDNYGIILDTKAYSSGYSLPIAQADEMERYVRENQTRDELVNPNQWWENFENGLGTFYFLFVAGHFNGNVQAQLERISRNTGVLGAAASISQLLLLADAIRGGRMDRERLRHLMFQNEEFLLEQEL

SEQ ID NO: 9 - protein, 201 aa, synthetic construct
  REGION 1..201: note = Synthetic Construct
VIEHEQTIKSSIEELKSELRTQLNVISHDYLQLVDISQDSQQNRLFEMKVMDLFINEFGYNGSHLGGSRKPDGILYTEGLSKDYGIIVDTKAYKDGYNLPIAQADEMERYIRENIDRNEVVNPNRWWEVFPSKINDYKFLFVSAYFKGNFKEQLERISINTGILGGAISVEHLLLGAEYFKRGILSLEDVRDKFCNTEIEF

SEQ ID NO: 10 - protein, 201 aa, synthetic construct
  REGION 1..201: note = Synthetic Construct
LQITQTLVDIEKERKKAYFLKETSLSPRYIELLEIAFDPKRNRDFEVITAELLKAGYGLKAKVLGGGRRPDGIAYTKDYGLIVDTKAYSNGYGKNIGQADEMIRYIEDNQKRDNKRNPIEWWREFEVQIPANSYYYLWVSGRFTGRFDEQLVYTSSQTNTRGGALEVEQLLWGADAVMKGKLNVSDLPKYMNNSIIKLTKK

SEQ ID NO: 11 - protein, 206 aa, synthetic construct
  REGION 1..206: note = Synthetic Construct
KLRFYEENITKETTDAIVVKDRARVRLHNINHKYLTLIDYAFSGKNNCTEFEIYTIDLLVNELAFNGIHLGGTRKPDGIFDYNQQGIIIDNKAYSKGFTITRSMADEMVRYVQENNDRNPERNKTQWWLNFGDNVNHFNFVFISSMFKSEVKHMLNNIKQSTGVDGCVLTAENLLYFADAIKGGTVKRTDFINLFGKNDELVYPYN

SEQ ID NO: 12 - protein, 201 aa, synthetic construct
  REGION 1..201: note = Synthetic Construct
LEITQELKDEQAEKRKAKFLKETNLPMKYIELLDIAYDGKRNRDFEIVTMELFRNVYRLHSKLLGGGRKPDGLLYQDRFGVIVDTKAYGKGYSKSINQADEMIRYIEDNKRRDENRNPIKWWEAFPDTIPQEEFYFMWVSSKFIGKFQEQLDYTSNETQIKGAALNVEQLLLGADLVLKGQLHISDLPSYFQNKEIEFVKA

SEQ ID NO: 13 - protein, 216 aa, synthetic construct
  REGION 1..216: note = Synthetic Construct
PRTKISKTNVLELKDKVRDKLKYVDHRYLALIDLAYDGTANRDFEIQTIDLLINELKFKGVRLGESRKPDGIISYNINGVIIDNKAYSTGYNLPINQADEMIRYIEENQTRDEKINSNKWWESFDDEVKDFNYLFVSSFFKGNFKNNLKHIANRTGVNGGAINVENLLYFAEELKAGRLSYVDSFTMYDNDEIYVGNIIDYSNLKIAADEEGLYSI

SEQ ID NO: 14 - protein, 175 aa, synthetic construct
  REGION 1..175: note = Synthetic Construct
MKYIELLDIAYDGKRNRDFEIVTMELFRNVYRLHSKLLGGGRKPDGLLYQDRFGVIVDTKAYGKGYSKSINQADEMIRYIEDNKRRDENRNPIKWWEAFPDTIPQEEFYFMWVSSKFIGKFQEQLDYTSNETQIKGAALNVEQLLLGADLVLKGQLHISDLPSYFQNKEIEFVKA

SEQ ID NO: 15 - protein, 197 aa, synthetic construct
  REGION 1..197: note = Synthetic Construct
VTDLNQIVKSSIEMSKANMRDNLQMLPHDYIELIEISQDPYQNRIFEMKVMDLFINEYGFSGSHLGGSRKPDGAMYAHGFGVIVDTKAYKDGYNLPISQADEMERYVRENIDRNEHVNSNRWWNIFPEDTNEYKFLFVSGFFKGNFEKQLERISIDTGVQGGALSVEHLLLGAEYIKRGILTLYDFKNSFLNKEIQF

SEQ ID NO: 16 - protein, 196 aa, synthetic construct
  REGION 1..196: note = Synthetic Construct
EASRSSVEELKSELRPQLRVLSHDYLQLVEIAQEPDQNRLFEMKVMELFVNELGFQGCHLGGSRRPDGILYTTDLEKNYGVIVDTKAYREGYSLPIGQADEMERYIRENIDRNPSVNPNKWWEAFPDDIENFTFLFVSGFFKGNFKDQLERISLNTGAAGGAISVEHLLLGADYYKRGVLTLEDFENHFCNGEIQF

SEQ ID NO: 17 - protein, 192 aa, synthetic construct
  REGION 1..192: note = Synthetic Construct
EVKKSSTEELKAQLRTQLTNISLDYLQLVDISTDSKQNRLFEMKVMDLFINELDFKGSHLGGGRKPDGAVYTTNYGIIVDTKAYKDGYNLPISQADEMERYVRENIDRNKGINPNEWWTIFPSSINDFTFLFVSGYFKGNFEGQLQRISMSTGIKGGAIGVEHLLLCAEYYKRGILSHQDIRDSFKNAEIEF

SEQ ID NO: 18 - protein, 198 aa, synthetic construct
  REGION 1..198: note = Synthetic Construct
SLAKSDFVETKERIRDKLLHLPHEYLSLIDLAYDSKQNRLFEMKTLGLLTEECGYHGLHLGGSRKPDGIIYTDTERYNYGVIIDTKAYSRGYNLPISQADEMERYIGENQTRDVKINPNKWWEYFPADVEEFYFMFVSGHFIGNFRSQIERISRNKAINGTAIAVANLLLCVEAYKAGELTHEAIKTKVFNNGEFELS

SEQ ID NO: 19 - protein, 193 aa, synthetic construct
  REGION 1..193: note = Synthetic Construct
PTARLEGRSELEYKKEEVRHQLTHLSHEYLGLLDLAYDSKQNRLFELKTMQLLTEECDFEGLHLGGSRKPDGIAYSESYGIIIDTKAYSGGYSLPISQADEMERYIGENQTRDPKVNPNEWWKNFSDTTQEFYFMFVAGHFKGKYQDQIERISCNKSVKGAAVSIEQLLLTVNAYKAGKLDHEGIKKALFESV

SEQ ID NO: 20 - protein, 198 aa, synthetic construct
  REGION 1..198: note = Synthetic Construct
NLAKSSLAEIKDEIRPQMTHLSHEYLSLIDLAYDSVQNRLFEMKTLELLTEECKFTGLHLGGSRKPDGIIYTNDLTENYGVIVDTKAYSKGYNLPISQADEMERYIRENQTRDKKINSNEWWLNFNTNIETYYFMFVAGHFIGNFVNQLERISMSTGVYGTALSVKNMLICANAIKSGDMCHEDMKNNMFHNSEYQII

SEQ ID NO: 21 - protein, 190 aa, synthetic construct
  REGION 1..190: note = Synthetic Construct
SLQKSSLSGMKDQIRARLTALPHEYLSLIDLAYDSEQNRLFEMKIIELFTEECGFSGRHLGGSNKPDGVISAADLSYGIIVDTKAYSKGYGLPLSQADEMERYVRENLTRDSRINPNEWWLAFDGAVPRFAFLFVSGHFTGTYGQRIERIIRSTGVPGAALAISKLLLYADTLKSGRISQQDFYRLVFPS

SEQ ID NO: 22 - protein, 200 aa, synthetic construct
  REGION 1..200: note = Synthetic Construct
PTARLEGKSEVEIIKEQMRGELTHLSHEYLGLLDLAYDSKQNRLFELKTMQLLTEECGFEGLHLGGSRKPDGIVYTKDESEQVDKENYGIIIDTKAYSGGYSLPISQADEMERYIGENQTRDIRINPNEWWKNFGDGVTEYYYLFVAGHFKGKYQEQIERINCNKSIKGAAVSIQQLLRIVNDYKAGKLTHEDMKLKLFY

SEQ ID NO: 23 - protein, 200 aa, synthetic construct
  REGION 1..200: note = Synthetic Construct
DLTRTDLLDVKEELREKLTHLSHEYLALIDLAYDSRQHRLFEMKTMELLIEECGYQGDHLGGSRRPDGICYTHNLYENYGIIIDTKAYKDGYNLPITQADEMERYIGDNAIRDTQRNPNKWWEHFSQDIRLFYFMFISGHFKGQYQDKINLLELNTGVCGAAIDIKKLLLTVNYYKAGIISHEDIASDFFQTTNDEADNS

SEQ ID NO: 24 - protein, 194 aa, synthetic construct
  REGION 1..194: note = Synthetic Construct
KAEKSEFLIEKDKLREKLDTLPHDYLSMVDLAYDSKQNRLFEMKTIELLINECNYKGLHLGGTRKPDGIVYTNNEVENYGIIIDTKAYSKGYNLPISQVDEMTRYVEENNKREKKRNPNEWWNNFDSDVKKFYFSFISGKFVGNIEEKLQRITLFTEIYGNAITVTTLLYIANEIKANRMKKSDIMEYFNDKVY

SEQ ID NO: 25 - protein, 213 aa, synthetic construct
  REGION 1..213: note = Synthetic Construct
KISKTNILELKDKVRDKLKYVDHRYLALIDLAYDGTANRDFEIQTIDLLINELKFKGVRLGESRKPDGIISYNINGVIIDNKAYSTGYNLPINQADEMIRYIEENQTRDEKINSNKWWESFDEKVKDFNYLFVSSFFKGNFKNNLKHIANRTGVNGGAINVENLLYFAEELKAGRISYLDSFKMYNNDEIYLGDISDYSYVKFAAEEEGEYLT

SEQ ID NO: 26 - protein, 201 aa, synthetic construct
  REGION 1..201: note = Synthetic Construct
PLEDSDIKNVKNRLMNKLPNLDPADFGLVDLAFAKAGTQSENTKMANEFEARTVEFMKQYFKLSGVHLGGGNRPDGALYDNDKYGIILDTKAYSQGYKPDTKQVREMSDYIQNVWYDSGRKEARAWWKNFPANLDKTSIHFIWVAGTFKSGMNDMIVAAKGHTAMTGGAITVEKLLTIADNVVAHNYNYDVLSDKFMDAVI

SEQ ID NO: 27 - protein, 206 aa, synthetic construct
  REGION 1..206: note = Synthetic Construct
SLQKSSLSGMKDQIRARLTALPHEYLSLIDLAYDSEQNRLFEMKIIELFTEECGFSGRHLGGSNKPDGVISAADLSYGIIVDTKAYSKGYGLPISQADEMERYVRENLTRDSRINPNEWWLAFDGAVPRFAFLFVSGHFTGTYGQRIERIIRSTGVPGAALEISKLLLYADALKSGRISQRDFYRLVFPPQPESEGLRRCPKPRKL

SEQ ID NO: 28 - protein, 192 aa, synthetic construct
  REGION 1..192: note = Synthetic Construct
EVVRSDIEETKAMLRENLKVLPHEYIELVEIAQDPDQNRVFEMKVIELFIKEYGFNGSHLGGSRRPDGAIFTDTFGVIVDTKAYKDGYNLPISQADEMERYVRENKERNEVANPNKWWSIFPETVKEYMFLFVSSFFKGNFRNHLERISLNTGVRGGVISVEHLLLGADYIKRGVLTLDDFRNKFNNDEIEF

SEQ ID NO: 29 - protein, 193 aa, synthetic construct
  REGION 1..193: note = Synthetic Construct
KVSKTNILELKDNTREKLVYLDHRYLSLFDLAYDDKASRDFEIQTIDLLINELQFKGLRLGERRKPDGIISYGVNGVIIDNKAYSKGYNLPIRQADEMIRYIQENQSRDEKLNPNKWWENFEEETSKFNYLFISSKFISGFKKNLQYIADRTGVNGGAINVENLLCFAEMLKSGKLEYNDFFNQYNNDEIIMR

SEQ ID NO: 30 - protein, 196 aa, synthetic construct
  REGION 1..196: note = Synthetic Construct
QLIKGEMENKKAELRQKLKHVPHEYIELIEIAQDSKQNRLLEFKVVEFFKKIYGYDGRHLGGSRKPDGALYTGSLKSNYGIILDTKAYKDGYSLPISQADEMQRYVDENNSRNQVINPNKWWEVYPISIVDFKFLFVSGFFKGEYKKQLERVSHLTKRKGAVLSIEQLLLGGEKIKDGSLTLVEVSDKFKNDAINF

SEQ ID NO: 31 - protein, 196 aa, synthetic construct
  REGION 1..196: note = Synthetic Construct
FLVKGAMEIKKSELRHKLRHVPHEYIELIEIAQDSKQNRLLEFKVVEFFKKIYGYRGKHLGGSRKPDGALFTDGLVLNHGIILDTKAYKDGYRLPISQADEMQRYVDENNKRSQVINPNEWWEIYPTSITDFKFLFVSGFFQGDYRKQLERVSHLTKCQGAVMSVEQLLLGGEKIKEGSLTLEEVGKKFKNDEIVF

SEQ ID NO: 32 - protein, 198 aa, synthetic construct
  REGION 1..198: note = Synthetic Construct
LPVKSEVSVFKDYLRTHLAHVDHRYLILVDLGFDGSSDRDYEMKTAELLTTELGFKGARLGDTRKPDVCVYHGNNGLIIDNKAYGKGYSLPIKQADEINRYIEENKERNELLNPNRWWNIFDHTVTHFRFAFISGSFTGGFKDRLNLISMRSGICGAAINSVNLLLMAEELKAGRLGYEEWFEAFDCNDEISFPLDLI

SEQ ID NO: 33 - protein, 144 aa, synthetic construct
  REGION 1..144: note = Synthetic Construct
PVLKDAALQKTKNTLLNELTEIDPADIEVIEMSWKKATTRSQNTLEATLFEVKVVEIFKKYFELNGEHLGGQNRPDGAVYYNSTYGIILDTKAYSNGYNIPVDQQREMVDYITDVIDKNQNVTPNRWWEAFPATLLKIIYIIYG

SEQ ID NO: 34 - protein, 196 aa, synthetic construct
  REGION 1..196: note = Synthetic Construct
VPVKSEVSLLKDYLRTHLLHVDHRYLILLDLGFDGTSDRDYEIQTAQLLTGELNFKGARLGDTRKPDVCVYYGEDGLIIDNKAYGKGYSLPIKQADEMYRYIEENKERNEKLNPNKWWEIFNNDVIHYHFAFISGAFTGGFKERLDNIRMRSGIYGAAVNSMNLLLMAEELKSGRLGYKECFKLFDCNDEIVLQRS

SEQ ID NO: 35 - protein, 190 aa, synthetic construct
  REGION 1..190: note = Synthetic Construct
PEADVERMLAKSFQHGALGMFIHEFAQMATESRKRATEFEQATASIFADVFGFQARHIGQAGAVERPDVVLASTSEHYGAILDSKAYASGYSARAGHRNTMRNYIERFADYALTEDPVAFFAYIVSDAKKTLNGQIKAIADQNGVPGSAITARDIIRMVERHQSGRPYTHQEIRDLLSNNRTLDYQDLNL

SEQ ID NO: 36 - protein, 196 aa, synthetic construct
  REGION 1..196: note = Synthetic Construct
VPVKSEVSLCKDYLRSYLTHVDHKYLILLDLGFDGTSDRDYEIQTAQLLTAELDFKGARLGDTRKPDVCVYYGEDGLIIDNKAYGKGYSLPIKQADEIYRYIEENKKRDEKLNPNKWWEIFDKGVVRYHFAFVSGAFTGGFKERLDNIRMRSGICGAAINSMNLLLMAEELKSGRLGYEECFALFDCNDEITFQSS

SEQ ID NO: 37 - protein, 193 aa, synthetic construct
  REGION 1..193: note = Synthetic Construct
GATKSDLSLLKDDIRKKLNHINHKYLVLIDLGFDGTADRDYELQTADLLTSELAFKGARLGDSRKPDVCVYHDKNGLIIDNKAYGSGYSLPIKQADEMLRYIEENQKRDKALNPNEWWTIFDDAVSKFNFAFVSGEFTGGFKDRLENISRRSYTNGAAINSVNLLLLAEEIKSGRISYGDAFTKFECNDEIII

SEQ ID NO: 38 - protein, 213 aa, synthetic construct
  REGION 1..213: note = Synthetic Construct
KISKTNVLELKDKVRDRLKYVDHRYLALIDLAYDGTANRDFEIQTIDLLINELKFKGVRLGESRKPDGIISYNINGVIIDNKAYSTGYNLPINQADEMIRYIEENQTRDEKINSNKWWESFDEKVKDFNYLFVSSFFKGNFKNNLKHIANRTGVNGGAINVENLLYFAEELKAGRLSYIDSFTMYDNDEIYVGNFSDYSYVKFAAEDQSDYRV

SEQ ID NO: 39 - protein, 222 aa, synthetic construct
  REGION 1..222: note = Synthetic Construct
NIAKSDFSIIKDNIRRKLQYVNHKYLLLIDLGFDSDSNRDYEIQTAELLTTELAFKGARLGDTRKPDVCVYYGENGLIIDNKAYSKGYSLPMSQADEMVRYIEENKARQSSINPNQWWKIFEDTVCNFNYAFVSGEFTGGFKDRLNNICERTRVSGGAINTINLLLLAEELKSGRMSYPKCFSYFDTNDEVHIPTYRDDDYEIHRSMAAEKSVEYGSQHGVN

SEQ ID NO: 40 - protein, 204 aa, synthetic construct
  REGION 1..204: note = Synthetic Construct
VLVKSEVSILKDYLRTHMIHVDHKYLILLDLGFDGTSDRDYEMQTAELLTKELAFQGARLGDTRKPDVCVYYGENGLIIDNKAYGKGYSLPMKQADEMYRYIEENKERSERFNKNKWWQIFDDQVKQFRFVFLSGSFTGGFKDRLNHISMRSGLNGAAISSVNLLLLAEELKSGRMRYEDCFKLFDGNDEVRLPGSFKRGGLMK

SEQ ID NO: 41 - protein, 193 aa, synthetic construct
  REGION 1..193: note = Synthetic Construct
VPVKSEVSICKDYLRSHLTHVDHKYLVLLDLGYDGNSDRDYEIQTAQLLTSELDFQGARLGDTRKPDVCVYYGKDGLIIDNKAYGKGYSLPIKQADEIYRYIEENKERNEMLNPNKWWEVFEESVTRYHFAFISGTFTGGFKDRLNNISMRSGICGAVINSMNLLLMAEALKSGRLSYEECFSLFDCNDEIIF

SEQ ID NO: 42 - protein, 199 aa, synthetic construct
  REGION 1..199: note = Synthetic Construct
KEIKNNINYVIDNTKNLDQNLIEKIIEQSFSGQKYCKEFEDSIFELYNKVIGFEGIKLGGVGNREPDSLMWYRASIDDDSYGLIVDAKAYSKGFRINTNSSRQMNDYIYTFANKLQDEYKINRSYYHWVSSKYVGNRDIENFAENVRNMYSFESKGSIVSISNALLLADRFQIHRDFKKLESLIAIQREILQKDIEILF

SEQ ID NO: 43 - protein, 201 aa, synthetic construct
  REGION 1..201: note = Synthetic Construct
IPVKSEVSVYKDYLRSRLTRIDHRYLILVDLGFDGNSDRDYEIQTAELLTKELSFQGARLGDTRKPDVCVFYGDKGLIIDNKAYGKGYSLPIKQADEMNRYLEENRERSDLLNPNRWWEIFDESVTHFRFAFLSGAFIGGFRDRLNLISVRNGLKGAAVSSVTLLLLAEELKSGRLKYEDFFLLFDCNDEISCPGLPEGLF

SEQ ID NO: 44 - protein, 198 aa, synthetic construct
  REGION 1..198: note = Synthetic Construct
ISVKSDMAVVKDSVRERLAHVSHEYLLLIDLGFDGTSDRDYEIQTAELLTRELDFLGGRLGDTRKPDVCIYYGKDGMIIDNKAYGKGYSLPIKQADEMYRYLEENKERNEKINPNRWWKVFDEGVTDYRFAFVSGSFTGGFKDRLENIHMRSGLCGGAIDSVTLLLLAEELKAGRMEYSEFFRLFDCNDEVTFQSIVI

SEQ ID NO: 45 - protein, 193 aa, synthetic construct
  REGION 1..193: note = Synthetic Construct
APVKSEVSVCKDYLRSRLTHVDHKYLLLLDLGYDGTSDRDYEIQTAGLLTDELDFKGARLGDTRKPDVCVYYGEDGLILDNKAYGKGYSLPIKQADEMYRYIEENKERNEMLNPNKWWEIFDRRVVRYHFAFVSGAFTGGFKERLNNIRMRSGICGAAVNSMNLLLMAEELKSGRLGYKECFALFDCNDEIVL

SEQ ID NO: 46 - protein, 192 aa, synthetic construct
  REGION 1..192: note = Synthetic Construct
PEEKSEVLLVKERVRSKLRALDPTYLRLVDLAYDGTADREFEISTIDLFTNELDFEGKHLGGSRKPDGIIYRDCNGLLIDNKAYSKGYSLPRAQVDEMGRYVRENKNRNAAINPLKWWENFPNSVTEFNFAFISSFFTGQYAERLSEIYHEYGVKGGVIDVENLLYIAEGLKSGDLSYSEFFELFDNSQILF

SEQ ID NO: 47 - protein, 201 aa, synthetic construct
  REGION 1..201: note = Synthetic Construct
EELRDKVIEEQKAIFLQKTKLPLSYIELLEIARDGKRSRDFELITMELFKNIYKINAIVLGGARKPDGVLYMPEFGVIVDTKAYADGYSKSIAQADEMIRYIEDNKRRDPSRNSTKWWEHFPTSIPANNFYFLWVSSVFVNKFHEQLSYTAQETQTVGAALSVEQLLLGADSVLKGNLTTKKFIDSFKNQEIVFAPSILHS

SEQ ID NO: 48 - protein, 197 aa, synthetic construct
  REGION 1..197: note = Synthetic Construct
NLTQELKDAALEEKKLKYQQLTKLPIKYIELLEIAYDGRRNRDFEILVADIFKNLYKFHSILLGGGRKPDGLIFTDKFGVIIDTKAYGEGYGKLITQEDEMVRYIEDNQQRDKNRNSITWWEKFNDAIPANSYYFMWVSSNFTGNFQEQLNSTSNRTGVKGAALNVEQLLLGAANAQQGILDISTFPSYMNNKEIIW

SEQ ID NO: 49 - protein, 197 aa, synthetic construct
  REGION 1..197: note = Synthetic Construct
KELKDEQSEKRKAYFLKETNLPLKYIELLDIAYDGKRNRDFEIVTMELFRNVYRLQSKLLGGVRKPDGLLYKHRFGIIVDTKAYGEGYSKSISQADEMIRYIEDNKRRDENRNSTKWWEHFPDCIPKQSFYFMWVSSKFVGKFQEQLDYTANETKTNGAALNVEQLLWGADLVAKGKLDISQLPSYFQNKEIEFVKA

SEQ ID NO: 50 - protein, 201 aa, synthetic construct
  REGION 1..201: note = Synthetic Construct
TELRDELIEQQKAIFLQKTKLPIEYIELLEIARDGNRSRDFEIITMGLFRDIYKINSTVLGGSRKPDGLLHMSDFGVIVDTKAYADGYSKNIAQADEMIRYIEDNKRRDSNRNPTKWWEIFPQTIPENKFYFLWISSSFVNKFPEQLNYTAQETQTVGAALNVEQLLLGADAILKNKLTIRKVVDSFKNQEIYFVPSILNN

SEQ ID NO: 51 - protein, 197 aa, synthetic construct
  REGION 1..197: note = Synthetic Construct
KELKNEQSEKLRSKFLKLTNLPMKYLELLDIAFDGKRNRDFEIVTMDLFRNVYKLNAKLLGGGRKPDGLIYTDGFGVIVDTKAYGEGYSKNINQADEMIRYIEDNKRRDLNRNPIEWWKDYPDSIPVDSFYFMWVSSKFVGKFQEQLEYTANETQTLGGALNVEQLLLGADLVAKGQFDAKELHSMFNNKEIVFDKV

SEQ ID NO: 52 - protein, 200 aa, synthetic construct
  REGION 1..200: note = Synthetic Construct
QLVPSYITQTKLRLSTLINYIDHSYFDLIDLGFDGRQNRLYELRIVELLNLISSLRALHLSGGNRPEIIAYSPDVNPINGVIMDSKSYRNGFNIPNSERDKMVRYIHEYNQKNPNLNSNKWWENFRVPNYPRSPIKYTFVSGNFISQFLSQIQYILTQTGINGGVITSEKLIKKVDTVLNPNISYTINDFFHELGCNGLV

SEQ ID NO: 53 - protein, 198 aa, synthetic construct
  REGION 1..198: note = Synthetic Construct
SPVKSEVSVFKDYLRTHLTHVDHRYLILVDLGFDGSSDRDYEMKTAELFTAELGFMGARLGDTRKPDVCVYHGAHGLIIDNKAYGKGYSLPIKQADEIYRYIEENKERAVRLNPNQWWKVFDESVAHFRFAFISGSFTGGFKDRIELISMRSGICGAAVNSVNLLLMAEELKSGRLNYEEWFQYFDCNDEISLPMSLT

SEQ ID NO: 54 - protein, 202 aa, synthetic construct
  REGION 1..202: note = Synthetic Construct
DEFKSSEADKIKTFLRPVLKHIDHHYLQAVDIAFKKNTSNQENTQFEILSTDLFTKEMGFHGRHLGGANKPDGFVYDQTDGWIIDSKAYSQGFAFTAHNTDAMSRYIRQYRTRNDKSTWWKDLPDNLPNTQFIYISSYFTGKYRQQLADYEHSNQMRGSLMEIAKLLMLAEKVKAGILNYNDFKKYALDKNTDFEFYSFILK

SEQ ID NO: 55 - protein, 200 aa, synthetic construct
  REGION 1..200: note = Synthetic Construct
RISPSNLEQTKQQLREELINLDHQYLDILDFSIAGNVGARQFEVRIVELLNEIIIAKHLSGGNRPEIIGFNPKENPEDCIIMDSKAYKEGFNIPANERDKMIRYVEEYNAKDNTLNNNEWWKNFESPNYPTNQVKFSFVSSSFIGQFTNQLTYINNRTNVNGSAITAETLLRKVENVMNVNTEYNLNNFFEELGSNTLVA

SEQ ID NO: 56 - protein, 197 aa, synthetic construct
  REGION 1..197: note = Synthetic Construct
KELKDEQSEKRKAKFLKETKLPMKYIELLDIAYDGKRNRDFEIVTMELFREVYRLNSKLLGGGRKPDGLIYTDDFGVIVDTKAYGEGYSKSINQADEMIRYIEDNKRRDEKRNPIKWWESFPSSISQNNFYFLWVSSKFVGKFQEQLAYTANETQTKGGAINVEQILIGADLIMQKMLDINAIPSFFENQEIIFKKV

SEQ ID NO: 57 - protein, 195 aa, synthetic construct
  REGION 1..195: note = Synthetic Construct
DILVDKEREMRKAKFLKETVLDSKFISLLDLAADATKSRDFEIVTAELFKEAYNLNSVLLGGSNKPDGLVFTDDFGILLDTKAYKNGFSIYAKDRDQMIRYVDDNNKRDKIRNPNEWWKSFSPLIPNDKFYYLWVSNFFKGQFKNQIEYVNRETNTYGAVLNVEQLLYGADAVIKGIINPNKLHEYFSNDEIKFK

SEQ ID NO: 58 - protein, 197 aa, synthetic construct
  REGION 1..197: note = Synthetic Construct
KELKNEQSEKRKAKFLKETDLPMKYIELLDIAYDGKRNRDFEIVTMELFRKVYKLHSKLLGGGRKPDGLIYKDDFGIIVDTKAYGEGYSKSIHQADEMIRYIEDNKRRDENRNPVKWWEHFPSIIPQDKFYFMWVSSKFVGKFQEQLDYTANETNTKGAALNVEQLLLGADLVSKGKLNATTLPSYFKNAEIEFIKA

SEQ ID NO: 59 - protein, 194 aa, synthetic construct
  REGION 1..194: note = Synthetic Construct
KELKDAALEHKKVQFQQLTQLPMKYIELLEIAYDGKRNRDFEILTADLFKYVYGFESILLGGGRKPDGLIFTDKFGVIIDTKAYSQGYGKSINQEDEMVRYIEDNQQRDETRNSVTWWDNFDDSIPDDSFYFLWVSSKFNGNFQEQLTSTHNRTGINGGAINVEQLLIGAAKVSKGQLDISTLPSYMDNKEIIW

SEQ ID NO: 60 - protein, 197 aa, synthetic construct
  REGION 1..197: note = Synthetic Construct
KELKDKASEQRKAEFMNKTDLPAKYIELLEIAFDGNRNRDFEIITAEIFKKVYGLKSVLLGGGRKPDCLVFNANFGMIIDTKAYSTGYSKSISQEDEMVRYIEDNQYRDTTRNPIEWWNNFPSSIKKEKYYFMWVSSKFIGRFQEQIESTYNRTNTKGAALNVEQLLLGANAVLRGELDANRISDYIDNKEILWVNN

SEQ ID NO: 61 - protein, 203 aa, synthetic construct
  REGION 1..203: note = Synthetic Construct
SCVKDEVNDIVDRVRVKLKNIDHKYLILISLAYSNETERTKKNSDARDFEIQTAELFTKELGFNGIRLGESNKPDVLISFGANGTIIDNKSYKDGFNIPRATSDQMIRYINENNQRTTQLNPNEWWKNFDSSVSNYTFLFVTSFLKGSFKNQIEYISNATNGTRGAAINVENLLYISEDIKSGIIKQSDFYSKFKNDEIVYPI

SEQ ID NO: 62 - protein, 195 aa, synthetic construct
  REGION 1..195: note = Synthetic Construct
KVQKSNILDVIEKCREKINNIPHEYLALIPMSFDENESTMFEIKTIELLTEHCKFDGLHCGGASKPDGLIYSEDYGVIIDTKSYKDGFNIQTPERDKMKRYIEENQNRNPQHNKTRWWDEFPHNISNFLFLFVSGKFGGNFKEQLRILSEQTNNTLGGALSSYVLLNIAEQIAINKIDHCDFKTRISCLDEVAFD

SEQ ID NO: 63 - protein, 202 aa, synthetic construct
  REGION 1..202: note = Synthetic Construct
AIRKEHITELKDKIRKKLHHISHSYLLLVDLAYSDADTKAKKNLEAKEFEIQTAKLFTKELDFSGSRLGDSNRPDVILSYGTQGTIIDNKSYKDGFNLDAGCRDEMSRYIEENQQRIPGVPSNEWWKSFDPSVTDFTFLFVTSYLKGNFKKGLSYISTMRKIQGACVNVENLLYLAENIKSGKTSYTEFFSLFNNEEIVIGS

SEQ ID NO: 64 - protein, 197 aa, synthetic construct
  REGION 1..197: note = Synthetic Construct
AEADVTSEKIKNHFRRVTELPERYLELLDIAFDHKRNRDFEMVTAGLFKDVYGLESVHLGGANKPDGVVYNDNFGIILDTKAYENGYGKHISQIDEMVRYIDDNRLRDTTRNPNKWWENFDADIPSDQFYYLWVSGKFLPNFAEQLKQTNYRSHANGGGLEVQQLLLGADAVKRRKLDVNTIPNYMKNEVITLVPEA

SEQ ID NO: 65 - protein, 211 aa, synthetic construct
  REGION 1..211: note = Synthetic Construct
LPQKDQVQQQQDELRPMLKNVDHRYLQLVELALDSDQNSEYSQFEQLTMELVLKHLDFDGKPLGGSNKPDGIAWDNDGNFIIFDTKAYNKGYSLAGNTDKVKRYIDDVRDRDTSRTSTWWQLVPKSIDVHNLLRFVYVSGNFTGNYMKLLDSLRSWSNAQGGLASVEKLLLTSELYLRNMYSHQELIDSWTDNNVKHDEYFLKIEKQLTIK

SEQ ID NO: 66 - protein, 170 aa, synthetic construct
  REGION 1..170: note = Synthetic Construct
MNFFSLHPNVYATGRPKGLIGMLENVWVSNHTPGEGTLYLISGFSNYNGGVRFYETFTEHINQGGRVIAILGGSTSQRLSSRQVVEELLNRGVEVHIINRKRILHAKLYGTSNNLGESLVVSSGNFTGPGMSQNIEASLLLDNNTTQSMGFSWNDMISEMLNQNWHIHNM

SEQ ID NO: 67 - protein, 194 aa, synthetic construct
  REGION 1..194: note = Synthetic Construct
ISVKSDMAVIKDSVRERLAHVSHEYLLLIDLGFDGTSDRDYEIQTAELLTRELDFLGGRLGDTRKPDVCIYYGKDGMIIDNKAYGKGYSLPIKQADEMYRYLEENKERNEKINPNRWWKVFDEGVTDYRFAFVSGSFTGGFKDRLENIHMRSGLCGGAMDSVTLLLLAEELKAGRMEYSEFFRLFDCNDEVTFR

SEQ ID NO: 68 - protein, 196 aa, synthetic construct
  REGION 1..196: note = Synthetic Construct
PLVKGEMEKKKSDLRHKLKHVPHEYIELIEIAQDSKQNRLFEFKVVEFLKEVYDYNGKHLGGSRKPDGALYTNGLKTDYGIILDTKAYKDGYSLPISQADEMQRYVDENNNRNAIINPNEWWKVYPNSILDFKFLFVSGFFKGDYKKQLARVSNLTKRKGAVLSVEQLLLGGEKIKDGSLTLEDVGDKFNNDEIIF

SEQ ID NO: 69 - protein, 136 aa, synthetic construct
  REGION 1..136: note = Synthetic Construct
PLVKGEMEKKKSDLRHKLKHVPHEYIELIEIAQDSKQNRLFEFKVVEFLKQVYDYNGKHLGGSRKPDGALYTNGLKTDYGIILDTKAYKDGYSLPISQADEMQRYVDENNNRNAIINPNEWWKVYPNSILDFKFLF

SEQ ID NO: 70 - protein, 197 aa, synthetic construct
  REGION 1..197: note = Synthetic Construct
SLAKSDLAESKEAVRAKLLNLSHEYLSLIDLAYDSKQNRLFEMKTLDLLIEECDYQGLHLGGSRKPDGIIYTITDKCKYGVIIDTKAYSKGYNLPISQADEMERYIGENQVRDEKVNPNMWWRNFDDEINEFYFMFVSGHFVGNYKAQIERISRTKGICGTALAVINLLLCAEAYKSGRLTHEDIKKEVFNNGEFVL

SEQ ID NO: 71 - protein, 199 aa, synthetic construct
  REGION 1..199: note = Synthetic Construct
DNVKSNISLLKDELRGQINHISHEYLSLVDLAFDSKQNRLFEMKVLELLVNEYGFKGKHLGGSRKPDGVVYSTTLEDNFGIIVDTKAYSGGYNLPISQADEMERYIRENTNRDEEVNPNKWWENFSEEVEKYYFVFISGSFKGKFEEQLKRLSMTTGVTGSAVNVVNLLLGAEKLKSGEFTIEELEKAMFNNSEFIVKY

SEQ ID NO: 72 - protein, 201 aa, synthetic construct
  REGION 1..201: note = Synthetic Construct
KLAKSSQSETKEKLREKLRNLPHEYLSLVDLAYDSKQNRLFEMKVIELLTEECGFQGLHLGGSRRPDGVLYTAGLTDNYGIILDTKAYSSGYSLPIAQADEMERYVRENQTRDELVNPNQWWENFENGLGTFYFLFVAGHFNGNVQAQLERISRNTGVLGAAASISQLLLLADAIRGGRMDRERLRHLMFQNEEFLLNQEL

SEQ ID NO: 73 - protein, 190 aa, synthetic construct
  REGION 1..190: note = Synthetic Construct
SLQKSSLSGMKDQIRARLTALPHEYLSLIDLAYDSEQNRLFEMKIIELFTEECGFSGRHLGGSNKPDGVISAADLSYGVIVDTKAYSKGYGLPLSQADEMERYVRENLTRDSRINPNEWWLAFDGAVPRFAFLFVSGHFTGTYGQRIERIIRSTGVPGAALAISKLLLYADELKSGRISQQDFYRLVFPS

SEQ ID NO: 74 - protein, 201 aa, synthetic construct
  REGION 1..201: note = Synthetic Construct
PHYKDLSEKSELSAEKEIVRAQLKNISHEYLSLMDIAFDSQQSRLFEMKFMELFLRECNFLGDHLGGASKPDGALYTDVYEGNYGIIVDTKAYSKGYDLPVNQRDEMLRYIRENHLRDKKQNPNEWWKIFPDNLNKFYFMFVSGKFKGGIAGKLEKIAAVHNVSGTAMPISTALLVAEKIKGGKMSMIEFANGIRNTEYEI

SEQ ID NO: 75 - protein, 198 aa, synthetic construct
  REGION 1..198: note = Synthetic Construct
KISKTNVLELKDKVRDKLKYVDNRYLALIDLAYDGTANRDFEIQTIDLLINELKFKGVRLGESRKPDGIISYDINGVIIDNKAYSSGYNLPINQADEMIRYIEENQTRDKKINPNKWWESFDDKVKDFNYLFVSSFFKGNFKNNLKHIANRTGVNGGVINVENLLYFAEELKSGRLSYVDLFKMYDNDEINIGNYCRL

SEQ ID NO: 76 - protein, 213 aa, synthetic construct
  REGION 1..213: note = Synthetic Construct
KISKTNVLELKDKVRDKLKYVDHRYLALIDLAYDGTANRDFEIQTIDLLINELKFKGVRLGESRKPDGIISYDINGVIIDNKAYSTGYNLPINQADEMIRYIEENQTRDKKINSNKWWESFDDKVKNFNYLFVSSFFKGNFKNNLKHIANRTGVNGGAINVENLLYFAEELKAGRLSYVDSFTMYDNDEIYVGNIIDYSNVKIAAEEESHYSI

SEQ ID NO: 77 - protein, 196 aa, synthetic construct
  REGION 1..196: note = Synthetic Construct
LTEKSELSAEKEILRAQLKNISHEYLSLMDIAFDSQQNRLFEMKFMELFLHECNFKGRHLGGASKPDGALYTDVYEGNYGIIVDTKAYSKGYDLPVSQRDEMLRYIRENSLRDKKQNPNEWWKIFPEELNKFYFMFVSGKFKGDIKGKLEKIAAVHNVNGTAMPIVTALLVAEKIRGGKMSMIEFARGIRNTEYEI

SEQ ID NO: 78 - protein, 213 aa, synthetic construct
  REGION 1..213: note = Synthetic Construct
KISKTNVLELKDKVRDKLKYVDHRYLALIDLAYDGTANRDFEIQTIDLLINELKFKGVRLGESRKPDGIISYNINGVIIDNKAYSTGYNLPINQADEMIRYIEENQTRDEKINSNKWWESFDDKVKDFNYLFVSSFFKGNFKNNLKHIANRTGVSGGAINVENLLYFAEELKAGRLSYVDSFKMYDNDEIYVGDFSDYSYVKFAAEEEGEYLT

SEQ ID NO: 79 - protein, 213 aa, synthetic construct
  REGION 1..213: note = Synthetic Construct
KISKTNVLELKDKVRNKLKYVDHRYLALIDLAYDGTANRDFEIQTIDLLINELKFKGVRLGESRKPDGIISYDINGVIIDNKSYSTGYNLPINQADEMIRYIEENQTRDEKINSNKWWESFDEKVKDFNYLFVSSFFKGNFKNNLKHIANRTGVNGGAINVENLLYFAEELKSGRLSYVDSFTMYDNDEIYVGSFTDYSNVKIAAEEESHYSI

SEQ ID NO: 80 - protein, 193 aa, synthetic construct
  REGION 1..193: note = Synthetic Construct
GAAKSDLSMLKDDIRKKLNHVNHKYLVLIDLGFDGTADRDYELQTADLLTSELAFKGARLGDSRKPDVCVYHDKNGLIIDNKAYGSGYSLPIKQADEMLRYIEENQKRDKALNPNEWWSIFDDAVSKFNFAFVSGEFTGGFKDRLENISRRSHTNGAAINSVNLLLLAEEIKSGRLTYGDALAKFECNDEILL

SEQ ID NO: 81 - protein, 197 aa, synthetic construct
  REGION 1..197: note = Synthetic Construct
KELKDEQSEKRKAKFLKETNLPMKYIELLDIAYDGKRNRDFEIVTMELFRKVYKLHSKLLGGGRKPDGLLYQDDFGVIVDTKAYGEGYSKSINQADEMIRYIEDNKRRDKNRNPIKWWEHFPSDIPQDKFYFMWVSSKFVGKFQEQLDYTANETNTKGAALNVEQLLLGADLVSKGELNTDTLPSYFKNTEIEFIKA

SEQ ID NO: 82 - protein, 194 aa, synthetic construct
  REGION 1..194: note = Synthetic Construct
SLRRKSLFLKYTLLPPEYIELLDIAYDGKRSRDFEIMTMELFKKIYGMNTVLLGGGRKPDGICFRSTFGIIVDTKAYSEGYSKNISQEDEMVRYITDNKLRDKARNPTQWWTAFPASIENYYFLWVSSRFIGKFAEQLTSTARETKTNGGALNVEQLLLGADMILKKELPPDSIANHFNNKEIFFADSIIDKHQ

SEQ ID NO: 83 - protein, 191 aa, synthetic construct
  REGION 1..191: note = Synthetic Construct
SVFKDYLRTHLTHVDHRYLILVDLGFDGSSDRDYEMKTAELFTAELGFMGARLGDTRKPDVCVYHGANGLIIDNKAYGKGYSLPIKQADEIYRYIEENKERDARLNPNQWWKVFDESVTHFRFAFISGSFTGGFKDRIELISMRSGICGAAVNSVNLLLMAEELKSGRLDYEEWFQYFDCNDEISFPVSLT

SEQ ID NO: 84 - protein, 197 aa, synthetic construct
  REGION 1..197: note = Synthetic Construct
KELRNEKFEQRRAKFLKITNLPMKYIELLEIAFDGARNRDFEILTMDLFRNIYKLPSKLLGGGRKPDGLVYTDKFGIIIDTKAYGEGYSKSINQADEMIRYIEDNKRRDVNRNPIEWWKEYPSSISNDSFYFLWISSQFVGKFQEQLDYTANETQTTGGALNVEQLLIGADLVAKGEFSSNELYSLFKNEEIIFKEV

SEQ ID NO: 85 - protein, 201 aa, synthetic construct
  REGION 1..201: note = Synthetic Construct
TELRDELIEQQKAIFLQKTKLPIEYIELLEIARDGNRSRDFEIVTMGLFRDIYKINSTVLGGSRKPDGLLHMSDFGVIVDTKAYADGYSKNIAQADEMIRYIEDNKRRDSNRNPTKWWEIFPQTIPENKFYFLWISSSFVNKFPEQLNYTAQETQTVGAALNVEQLLLGADAILKNKLTIRKVVDSFKNQEIYFVPSILNN

SEQ ID NO: 86 - protein, 197 aa, synthetic construct
  REGION 1..197: note = Synthetic Construct
QELKDEQAEKRKAKFLKETNLPMKYIELLDIAYDGKRNRDFEIVTMELFRNVYRLHSKLLGGGRKPDGLLYQDCFGVIVDTKAYGKGYSKSINQADEMIRYIEDNKRRDENRNPIKWWEAFPDKIPQEEFYFMWVSSKFIGKFQEQLDYTSNETQIKGAALNVEQLLLGADLVLKGQLHISDLPSYFQNKEIEFVKA

SEQ ID NO: 87 - protein, 201 aa, synthetic construct
  REGION 1..201: note = Synthetic Construct
EELRDKVIEEQKAIFLQKTKLPLSYIELLEIARDGKRSRDFELITMELFRDIYKIKAIVLGGARKPDGVLYMPEFGVIVDTKAYADGYSKSIAQADEMIRYIEDNKRRDPSRNSTKWWEHFPTSIPANNFYFLWVSSVFVNKFHEQLSYTAQETQTVGAALSVEQLLLGADSVLKGNLTTEKFIDSFKNQEIVFAPSILHS

SEQ ID NO: 88 - protein, 194 aa, synthetic construct
  REGION 1..194: note = Synthetic Construct
AELKDKAADAVKAKFLKLTGLSMKYIELLDIAYDSSRNRDFEILTADLFKNVYGLDAMHLGGGRKPDAIAQTSHFGIIIDTKAYSNGYSKSISQEDEMVRYIEDNQQRSITRNSVEWWKNFNSSIPSTAFYFLWVSSKFVGKFDDQLLSTYNRTNTCGGALNVEQLLIGAYKVKAGLLGIGQIPSYFKNKEIAW

SEQ ID NO: 89 - protein, 194 aa, synthetic construct
  REGION 1..194: note = Synthetic Construct
AELKDKAADAVKAKFLKLTGLSMKYIELLDIAYDSSRNRDFEILTADLFKNVYGLDAMHLGGGRKPDAIAQTSHFGIIIDTKAYGNGYSKSISQEDEMVRYIEDNQQRSITRNSVEWWKNFNSSIPSTAFYFLWVSSKFVGKFDDQLLATYNRTNTCGGALNVEQLLIGAYKVKAGLLGIGQIPSYFKNKEIAW

SEQ ID NO: 90 - protein, 197 aa, synthetic construct
  REGION 1..197: note = Synthetic Construct
QELKDEKAEQRKAKFLKETNLSMKYIELLDIAYDGKRDRDFEIVTMELFRKVYKLKSKLLGGGRKPDGLVYSDEFGIIVDTKAYGNGYPKSISQADEMIRYIEDNKRRDEKRNSTKWWEYFSSVIPDDSFYFMWISSKFIGKFQEQLIYTANETEINGAALNVEQLLIGADKILKGELSVNKLPNYFINQEIIFEKT

SEQ ID NO: 91 - protein, 199 aa, synthetic construct
  REGION 1..199: note = Synthetic Construct
NELRNAALDKQKVNFINKTGLPMKYIELLEIAFDGSRNRDFEMVTADLFKNVYGFNSILLGGGRKPDGLIFTDRFGVIIDTKAYGNGYSKSIGQEDEMVRYIEDNQLRDSNRNSVEWWKNFDEKIESENFYFMWISSKFIGQFSDQLQSTSDRTNTKGAALNVEQLLLGAAAARDGKLDINSLPIYMNNKEILWSGDFS

SEQ ID NO: 92 - protein, 196 aa, synthetic construct
  REGION 1..196: note = Synthetic Construct
KELRNEVAEERRAYFLKNTNLPTKYIELLDIAYDGKRNRDFEILTMDLFRNVYKLNSKLLGGGRKPDGLVYSNQFGIIVDTKAYSEGYSKSIQQADEMIRYIEDNKRRDINRNPIEWWKDFPNSIKDDSYYFLWVSSKFVGKFPEQLTYTANQTETIGGALNVEQLLLGADKVKKGEIQSDKLNTYFENKEIIFQS

SEQ ID NO: 93 - protein, 201 aa, synthetic construct
  REGION 1..201: note = Synthetic Construct
EELRDKVIEEQKAIFLQKTKLPLSYIELLEIARDGKRSRDFELITMELFKNIYKINAIVLGGARKPDGVLYMPEFGVIVDTKAYADGYSKSIAQADEMIRYIEDNKRRDPSRNSTKWWEHFPTSIPANNFYFLWVSSVFVNKFHEQLSYTAQETQTVGAALSVEQLLLGADSVLKGNLTTEKFIDSFKNQEIVFAPSILHS

SEQ ID NO: 94 - protein, 201 aa, synthetic construct
  REGION 1..201: note = Synthetic Construct
EELRDKVIEEQKAIFLQKTKLPLSYIELLEIARDGKRSRDFELITMELFKNIYKINASILGGARKPDGVLYMPEFGVIVDTKAYADGYSKSIAQADEMIRYIEDNKRRDPSRNSTKWWEHFPTSIPANNFYFLWVSSVFVNKFHEQLSYTAQETQTVGAALSVEQLLLGADSVLKGNLTTEKFIDSFKNQEIVFAPSILHS

SEQ ID NO: 95 - protein, 194 aa, synthetic construct
  REGION 1..194: note = Synthetic Construct
QELKDAALEEKKLKYQQLTKLPIKYIELLEIAYDGRRNRDFEILVADIFKNIYKFHSILLGGGRKPDGLIFTDKFGVIIDTKAYGEGYGKLITQEDEMVRYIEDNQQRDKNRNSITWWEKFNDAIPANSYYFMWVSSNFTGNFQEQLNSTSNRTGVKGAALNVEQLLLGAANAQQGILDISTFPSYMNNKEIIW

SEQ ID NO: 96 - protein, 201 aa, synthetic construct
  REGION 1..201: note = Synthetic Construct
EELRDKVIEEQKAIFLQKTKLPLSYIELLEIARDGKRSRDFEFITMELFKNIYKINARILGGARKPDGVLYMPEFGVIVDTKAYADGYSKSIAQADEMIRYIEDNKRRDPSRNSTKWWEHFPTSIPANNFYFLWVSSVFVNKFHEQLSYTAQETQTVGAALSVEQLLLGADSVLKGNLTTEKFIDSFKNQEIVFAPSILHS

SEQ ID NO: 97 - protein, 211 aa, synthetic construct
  REGION 1..211: note = Synthetic Construct
DSINDFDIPNLQITQTLVDIEKERKKAYFLKETSLSPRYIELLEIAFDPKRNRDFEVITAELLKAGYGLKAKVLGGGRRPDGIAYTKDYGLIVDTKAYSNGYGKNIGQADEMIRYIEDNQKRDNKRNPIEWWREFEVQIPANSYYYLWVSGRFTGRFDEQLVYTSSQTNTRGGALEVEQLLWGADAVMKGKLNVSDLPKYMNNSIIKLTKK

SEQ ID NO: 98 - protein, 201 aa, synthetic construct
  REGION 1..201: note = Synthetic Construct
EELRDKVIEEQKAIFLQKTKLPLSYIELLEIARDGKRSRDFELITMELFKNIYKINASILGGARKPDGVLYMPEFGVIVDTKSYADGYSKSIAQADEMIRYIEDNKRRDPSRNSTKWWEHFPTSIPANNFYFLWVSSVFVNKFHEQLSYTAQETQTVGAALSVEQLLLGADSVLKGNLTTEKFIDSFKNQEIVFAPSILHS

SEQ ID NO: 99 - protein, 198 aa, synthetic construct
  REGION 1..198: note = Synthetic Construct
ISVKSDMAVVKDSVRERLAHVSHEYLILIDLGFDGTSDRDYEIQTAELFTRELDFLGGRLGDTRKPDVCIYYGKDGMIIDNKAYGKGYSLPIKQADEMYRYLEENKERNEKINPNRWWKVFDEGVTDYRFAFVSGSFTGGFKDRLENIHMRSGLCGGAIDSVTLLLLAEELKAGRMEYSEFFRLFDCNDEVTFQSIVI

SEQ ID NO: 100 - protein, 197 aa, synthetic construct
  REGION 1..197: note = Synthetic Construct
KELKDKASEQRKAEFMNKTDLPAKYIELLEIAFDGNRNRDFEIITAEIFKKVYGLKSVLLGGGRKPDCLVFNANFGMIIDTKAYSTGYSKSISQEDEMVRYIEDNQYRDTTRNPIEWWNNFPSSIKKEKYYFMWVSSKFIGRFQEQIESTYNRTNTKGAALNVEQLLLGANAVLRGELDANRISDYIDNKEILWFNN

SEQ ID NO: 101 - protein, 198 aa, synthetic construct
  REGION 1..198: note = Synthetic Construct
TQTLVDIEKERKKAYFLKETSLSPRYIELLEIAFDPKRNRDFEVITAELLKAGYGLKAKVLGGGRRPDGIAYTKDYGLIVDTKAYSNGYGKNIGQADEMIRYIEDNQKRDSKRNPIEWWREFEVQIPANSYYYLWVSGRFTGRFDEQLVYTSSQTNTRGGALEVEQLLWGADAVMKGKLNVSDLPKYMNNSIIKLTKK

SEQ ID NO: 102 - protein, 198 aa, synthetic construct
  REGION 1..198: note = Synthetic Construct
NLDKVERDSRKAEFLAKTSLPPRFIELLSIAYESKSNRDFEMITAEFFKDVYGLGAVHLGNARKPDALAFTDNFGIVIDTKAYSNGYSKNINQEDEMVRYIEDNQIRSPERNKNEWWLSFPPSIPENNFHFLWVSSYFTGYFEEQLQETSDRAGGMTGGALDIEQLLIGGSLVQEGKLAPHDIPEYMQNRVIHFGDLN

SEQ ID NO: 103 - protein, 198 aa, synthetic construct
  REGION 1..198: note = Synthetic Construct
NLDNVERDNRKAEFLAKTSLPPRFIELLSIAYESKSNRDFEMITAELFKDVYGLGAVHLGNAKKPDALAFNDDFGIIIDTKAYSNGYSKNINQEDEMVRYIEDNQIRSPDRNNNEWWLSFPPSIPENDFHFLWVSSYFTGRFEEQLQETSARTGGTTGGALDVEQLLIGGSLIQEGSLAPHEVPAYMQNRVIHFGDLN

SEQ ID NO: 104 - protein, 194 aa, synthetic construct
  REGION 1..194: note = Synthetic Construct
ISVKSDMAVVKDSVRERLAHVSHEYLLLIDLGFDGTSDRDYEIQTAELLTRELDFLGGRLGDTRKPDVCIYYGKDGMIIDNKAYGKGYSLPIKQADEMYRYLEENKERNEKINPNRWWKVFDEGVTDYRFAFVSGSFTGGFKDRLENIHMRSGLCGGAIDSVTLLLLAEELKAGRMEYSEFFRLFDCNDEVIFR

SEQ ID NO: 105 - protein, 194 aa, synthetic construct
  REGION 1..194: note = Synthetic Construct
ISVKSDMAVVKDSVRERLAHVSHEYLLLIDLGFDGTSDRDYEIQTAELLTRELDFLGGRLGDTRKPDVCIYYGKDGMIIDNKAYGKGYSLPIKQADEMYRYLEENKERNEKINPNRWWKVFDEGVTDYRFAFVSGSFTGGFKDRLENIHMRSGLCGGAIDSVTLLLLAEELKAGRMEYSEFFRLFDCNDEVTFR

SEQ ID NO: 106 - protein, 198 aa, synthetic construct
  REGION 1..198: note = Synthetic Construct
TQTLVDIEKERKKAYFLKETSLSPRYIELLEIAFDPKRNRDFEVITAELLKAGYGLKAKVLGGGRRPDGIAYTKDYGLIVDTKAYSNGYGKNIGQADKMIRYIEDNQKRDSKRNPIEWWREFEVQIPANSYYYLWVSGRFTGRFDEQLVYTSSQTNTRGGALEVEQLLWGADAVMKGKLNVSDLPKYMNNSIIKLTKK

SEQ ID NO: 107 - protein, 194 aa, synthetic construct
  REGION 1..194: note = Synthetic Construct
ISVKSDMAVIKDSVRGRLAHVSHEYLLLIDLGFDGTSDRDYEIQTAELLTRELDFLGGRLGDTRKPDVCIYYGKDGMIIDNKAYGKGYSLPIKQADEMYRYLEENKERNEKINPNRWWKVFDEGVTDYRFAFVSGSFTGGFKDRLENIHMRSGLCGGAMDSVTLLLLAEELKAGRMEYSEFFRLFDCNDEVTFR

SEQ ID NO: 108 - protein, 194 aa, synthetic construct
  REGION 1..194: note = Synthetic Construct
QELKDKYSDALKAKYIKLTGLPMKYIELLDIAFDGKRNRDFEIITADLFKNIYGLESVLLGGGRKPDGIIFTDKFGVIVDTKAYGNGYSKEIKQEDEMVRYIEDNQLRDKERNPVEWWNNFNPSIPSNSFYFMWISSKFIGKFTEQLESTYNRTGVHGGALNVEQLLLGAHKVQIGELDVHHLPDYIQNKEIFW

SEQ ID NO: 109 - protein, 199 aa, synthetic construct
  REGION 1..199: note = Synthetic Construct
KITKSDLTVVKDQIRKQLVHIDHKYLVLIDLGFDGRANRDYEIQTAELLTGELEFKGTRLGDTRKPDVCVYYGKDGLIIDNKAYGKGYSLPISQADEMVRYLEENKTRQTAVNPNEWWNIFEDSVKDFHFAFVSGEFVGGFQDKLQNIYERTGVRGAAMNTANLLLFAEELKAGRLEYSDCFSYFDGNEEIRDFYIWNQ

SEQ ID NO: 110 - protein, 200 aa, synthetic construct
  REGION 1..200: note = Synthetic Construct
QLTQSQGDKAREQLKAKFLAKTNLLPRYVELLDIAYDSKRNRDFEMVTAELFNFAYLLPAVHLGGVRKPDALVATKKFGIIVDTKAYANGYSRNANQADEMARYITENQKRDPKTNPNRWWDNFDARIPPNAYYFLWVSSFFTGQFDDQLSYTAHRTNTHGGALNVEQLLIGANMIQTGQLDRNKLPEYMQDKEITFGTI

SEQ ID NO: 111 - protein, 204 aa, synthetic construct
  REGION 1..204: note = Synthetic Construct
LPVKSQVSILKDYLRSYLSHVDHKYLILLDLGFDGTSDRDYEIWTAQLLTAELSFLGGRLGDTRKPDVCIYYEDNGLIIDNKAYGKGYSLPIKQADEMYRYIEENKERSELLNPNCWWNIFGEGVKTFRFAFLSGEFTGGFKDRLNHISMRSGIKGAAVNSANLLIMAEQLKSGTMSYEEFFQLFDHNDEIIFPHLSLQGGLIL

SEQ ID NO: 112 - protein, 204 aa, synthetic construct
  REGION 1..204: note = Synthetic Construct
LPVKSQVSILKDYLRSCLSHVDHKYLILLDLGFDGTSDRDYEIQTAQLLTAELSFLGGRLGDTRKPDVCIYYEDNGLIIDNKAYGKGYSLPIKQADEMYRYIEENKERSELLNPNCWWNIFDEGVKTFRFAFLSGEFTGGFKDRLNHISMRSGIKGAAVNSANLLIMAEQLKSGTMSYEEFFQLFDHNDEIIFPHLSIQGGLIL

SEQ ID NO: 113 - protein, 196 aa, synthetic construct
  REGION 1..196: note = Synthetic Construct
QELKDLETERRKAEFMNKTDLSAKYIELLEIAYDGKRNRDFEIVTAELFKKVYGLQSILLGGGRKPDAIVFTDKFGFIIDTKAYGEGYSKSISQADEMIRYIEDNKRRDINRNPTEWWIDFDPIIPQNQFYFMWVSSKFVGRFQEQLDYTASQTSTNGGALNVEQLLLGADAVLKGILDANTLPLYMKNKEIEFIS

SEQ ID NO: 114 - protein, 201 aa, synthetic construct
  REGION 1..201: note = Synthetic Construct
QIAKDTTDTVAVKNRARLRLHNIDHKYLTLIDYAFSGKDKCIDFEVYTIDLLVNELAFNGVHLGGTRKPDGIFYHNNNGVIIDNKAYSKGFTISRGMADEMTRYVQENNDRNPERNPNQWWLNFSDNVNHFNFVFISSLFKGNIELMLNNIKQSTGVEGCALTVENLLYFADAIKGGDMHKDAFIDQFGAGKEIVCTIYRT

SEQ ID NO: 115 - protein, 196 aa, synthetic construct
  REGION 1..196: note = Synthetic Construct
LPMKSEVSILKDYLRSHLTYIDHKYLILVDLGYDGTSDRDYEIQTAQLLTAELSFLGGRLGDTRKPDVCIYYENNGLIIDNKAYGKGYSLPIKQADEMYRYIEENKERSELLNPNCWWNIFGKDVKNFRFAFLSGEFTGGFRDRLNHISMRSGMKGAAVNSANLLIMAEKLKAGIMGYEEFFRLFDTNDEIIFLHE

SEQ ID NO: 116 - protein, 204 aa, synthetic construct
  REGION 1..204: note = Synthetic Construct
LPVKSQVSILKDYLRSYLSHVDHKYLILLDLGFDGTSDRDYEIQTAQLLTAELSFVGGRLGDTRKPDVCIYYEDNGLIIDNKAYGKGYSLPIKQADEMYRYIEENKERSELLNPNCWWNIFDEGVKTFHFAFLSGEFTGGFKDRLNHISMRSGIKGAAVNSANLLIMAEQLKSGTMSYEEFFQLFDHNDEIIFPHLSLQGGLIL

SEQ ID NO: 117 - protein, 195 aa, synthetic construct
  REGION 1..195: note = Synthetic Construct
LTSKEKSNLKLKEFFISETAIPNKFITLFDLAYDGSANRDFEIITSELFRDVYKLNTKHLGGTRKPDILIWNKEYGIIADTKAYSKGYKKNISEEDKMVRYIDENIKRNKNDNPNEWWKIFDKNISSANYFYLWISSEFVGKFEEQLQGTVTRTNTNGASLNVYQLLMGAHLVQIEELSVNSIPAYMNNMEIKFV

SEQ ID NO: 118 - protein, 197 aa, synthetic construct
  REGION 1..197: note = Synthetic Construct
LPVKSEVSILKDYLRSHLTHIDHKYLILVDLGYDGTSDRDYEIQTAQLLTAELSFLGGRLGDTRKPDVCIYYEDNGLIIDNKAYGKGYSLPIKQADEMYRYIEENKERSQLLNPNCWWDIFGKDVKTFHFAFVSGEFTGGFRDRLNHISMRSGLKGAAVNSANLLIMAEKLKAGTMEYGEFFRFFDTNDEILFLHES

SEQ ID NO: 119 - protein, 195 aa, synthetic construct
  REGION 1..195: note = Synthetic Construct
LSNNDKQRLKLKEYFIQNTNLPAKFITLLDIAYDGQANRDFEIITTELFRDVYKLKAQHMGGTRKPDALIWTSQFGVIVDTKAYSKGYKKNISEADKMVRYVNENIERNKKSNPNEWWKSFDSSIPSNQYYYLWISSEFIGRFDEQLKETTSRTRTNGAALNVYQLLSGADLVQKNNLDSNNLPSYINNTEIKFV

SEQ ID NO: 120 - protein, 204 aa, synthetic construct
  REGION 1..204: note = Synthetic Construct
LPVKSQVSILKDYLRSYLSHVDHKYLILLDLGFDGTSDRDYEIQTAQLLTAELSFLGGRLGDTRKPDVCIYYEDNGLIIDNKAYGKGYSLPIKQADEMYRYIEENKERSELLNPNCWWNIFDEGVKTFRFAFLSGEFTGGFKDRLNLISMRSGIKGAAVNSANLLIMAEQLKSGTMSYEEFFQLFDHNDEIIFPHLSLQGGLIL

SEQ ID NO: 121 - protein, 203 aa, synthetic construct
  REGION 1..203: note = Synthetic Construct
ECVKDNVVDIKDRVRNKLIHLDHKYLALIDLAYSDAASRAKKNADAREFEIQTADLFTKELSFNGQRLGDSRKPDVIISYGLDGTIVDNKSYKDGFNISRTCADEMSRYINENNLRQKSLNPNEWWKNFDSTITAYTFLFITSYLKGQFEDQLEYVSNANGGIKGAAIGVESLLYLSEGIKAGRISHADFYSNFNNKEMIYTA

SEQ ID NO: 122 - protein, 196 aa, synthetic construct
  REGION 1..196: note = Synthetic Construct
VPVKSEVSLLKDYLRSHLLHVDHRYLVLLDLGFDGTSDRDYEIQTAQLLTGELNFKGARLGDTRKPDVCVYYGEDGLIIDNKAYGKGYSLPIKQADEMYRYIEENKERNEKLNPNKWWEIFDNNVIHYHFAFVSGAFTGGFKERLDNIRMRSGIYGAAVNSMNLLLMAEELKSGRLGYKECFKLFDCNDEIVLQRS

SEQ ID NO: 123 - protein, 193 aa, synthetic construct
  REGION 1..193: note = Synthetic Construct
NEEKDKLKVKEFFISETSIPNKFITLLDLAYDGNANRDFEIITSEFIREVYKLNTKHLGGTRKPDILIWNDEFGIIADTKAYSKGYKKNISEEDKMVRYIDENAKRSKDDNPNEWWINFGKNIPSSNYFYLWVSSEFIGKFEEQLKETASRTNTNGASLNVYQLLMGGHLVQTGRFNISNLPAYMNNSEIKFS

SEQ ID NO: 124 - protein, 197 aa, synthetic construct
  REGION 1..197: note = Synthetic Construct
NALKDKHLEKIKEKFLENTSLDPRFISLIEISRDKKQNRAFEIITAELFNTSYKLSATHLGGGRRPDVLVYNDNFGIIVDTKAYKDGYGRNVNQEDEMVRYITENNIRKQDINKNDWWKYFSKSIPSTSYYHLWISSQFVGMFSDQLRETSSRTGENGGAMNVEQLLIGANQVLNNVLDPNCLPKYMENKEIIFETL

SEQ ID NO: 125 - protein, 196 aa, synthetic construct
  REGION 1..196: note = Synthetic Construct
LPVKSEVSILKDYLRSHLTNIDHKYLILVDLGYDGTSDRDYEIQTAQLLTAELSFHGGRLGDTRKPDVCIYYEDNGLIIDNKAYGKGYSLPIKQADEMYRYIEENKERSELLNPNCWWNIFGKDVKTYHFAFLSGEFTGGFRDRLNNISMRSGIKGAAVNSANLLILAERLKSGTMRYEEFFRLFDTNDEILFLHE

SEQ ID NO: 126 - protein, 196 aa, synthetic construct
  REGION 1..196: note = Synthetic Construct
VPVKSEMSLLKDYLRTHLLHVDHRYLILLDLGFDGASDRDYEIQTAQLLTGELNFKGARLGDTRKPDVCVYYGEDGLIIDNKAYGKGYSLPIKQADEMYRYIEENKERNEKLNPNKWWEIFDNDVIHYHFAFVSGAFTGGFKERLDNIRMRSGIYGAAVNSMNLLLMAEELKSGRLGYKECFKLFDCNDEIVLQRS

SEQ ID NO: 127 - protein, 198 aa, synthetic construct
  REGION 1..198: note = Synthetic Construct
NLKLRTEEKERLELKEYFISNTDIPSKYITLLDLAYDGNANRDFEIVTAELFKDVFQLKTKHLGGTRKPDILIWTDKFGVIADTKAYSKGYKKNISEADKMVRYVNENTNRNKNDNSNEWWNSFETKIPANAYYFLWISSKFIGKFNEQLIETSSRTGRNGAAIDVYQLLRGADLVQKSKFNVHDLPSLMQNKEIQFI

SEQ ID NO: 128 - protein, 196 aa, synthetic construct
  REGION 1..196: note = Synthetic Construct
VPVKSEVSLLKDYLRTHLLHVDHRYLILLDLGFDGTSDRDYEIQTAQLLTGELNFKGARLGDTRKPDVCVYYGEDGLIIDNKAYGKGYSLPIKQADEMYRYIEENKERNEKLNPNKWWEIFDNDVIHYHFAFISGAFTGGFKERLDNIRMRSGIYGAAVNSMNLLLMAEELKSGRLGYKECFKLFDCNDEIVLQRS

SEQ ID NO: 129 - protein, 203 aa, synthetic construct
  REGION 1..203: note = Synthetic Construct
SCVKDEVNDIVDRVRVKLKNIDHKYLILISLAYSDETERTKKNSDARDFEIQTAELFTKELGFNGIRLGESNKPDVLISFGANGTIIDNKSYKDGFNIPRVTSDQMIRYINENNQRTTQLNPNEWWKNFDSSVSNYTFLFVTSFLKGSFKNQIEYISNATNGTRGAAINVESLLYISEDIKSGKIKQSDFYSEFKNDEIVYPI

SEQ ID NO: 130 - protein, 196 aa, synthetic construct
  REGION 1..196: note = Synthetic Construct
APVKSEVSLCKDILRSHLTHVDHKYLILLDLGFDGTSDRDYEIQTAQLLTAELDFKGARLGDTRKPDVCVYYGEDGLILDNKAYGKGYSLPIKQADEMYRYIEENKERNERLNPNKWWEIFDKDVVRYHFAFVSGTFTGGFKERLDNIRMRSGICGAAVNSMNLLLMAEELKSGRLGYKECFALFDCNDEIAFQCS

SEQ ID NO: 131 - protein, 196 aa, synthetic construct
  REGION 1..196: note = Synthetic Construct
VPVKSEVSLCKDYLRSHLNHVDHRYLILLDLGFDGTSDRDYEIQTAQLLTGELNFKGARLGDTRKPDVCVYYGEDGLIIDNKAYGKGYSLPIKQADEMYRYIEENKERNEKLNPNKWWEIFDKDVIHYHFAFVSGAFTGGFKERLENIRMRSGIYGAAVNSMNLLLMAEELKSGRLDYKECFKLFDCNDEIVLQRS

SEQ ID NO: 132 - protein, 195 aa, synthetic construct
  REGION 1..195: note = Synthetic Construct
LTSKEKNNLELKEFFVSNTNIPSKFISLLDLAYDGSVSRDFEIVTSELFREVYKLNTKHLGGTRKPDILIWNEDFGIITDTKAYSKGYKKNISEEDKMVRYIDENIKRSKSDNQNEWWNIFDKNISSTNFFYLWISSEFIGKFEEQLHETASRTNTNGASLNVYQLLMGAHLVQTGKIDISNIPSFMNNEEIKFV

SEQ ID NO: 133 - protein, 203 aa, synthetic construct
  REGION 1..203: note = Synthetic Construct
SCVKDEVNDIVDRVRVKLKHVDHKYLILISLAYSNETERTKKNSDARDFEIQTAELFTKELGFNGIRLGESNKPDVLISFGANGTIIDNKSYKDGFNIPRATSDQMIRYINENNQRTTQLNPNEWWKNFDSSVLNYTFLFVTSFLKGSFKNQIEYISKATNGTRGAAINVENLLYISEDIKSGNIKQSDFYSEFKNDEIVYSI

SEQ ID NO: 134 - protein, 196 aa, synthetic construct
  REGION 1..196: note = Synthetic Construct
VPVKSEVSLCKDYLRSHLNHVDHKYLILLDLGFDGTSDRDYEIQTAQLLTGELNFKGARLGDTRKPDVCVYYGEDGLIIDNKAYGKGYSLPIKQADEMYRYIEENKERNEKLNPNKWWEIFDNDVIHYHFAFVSGAFTGGFRERLENIRMRSGIYGAAVNSMNLLLMAEELKSGRLGYKECFKLFDCNDEIVLQRS

SEQ ID NO: 135 - protein, 197 aa, synthetic construct
  REGION 1..197: note = Synthetic Construct
NVLKDKHLEKIKEKFLENTSLDPRFISLIEISRDKKQNRAFEIITAELFNTSYNLSAIHLGGGRRPDVLVYNDNFGIIVDTKAYKDGYGRNVNQEDEMVRYITENNIRKQDISKNNWWKYFSKSIPSTSYYHLWISSEFVGMFSDQLRETSSRTGENGGAMNVEQLLIGANQVLNNVLDPNRLPEYMENKEIIFGTL

SEQ ID NO: 136 - protein, 196 aa, synthetic construct
  REGION 1..196: note = Synthetic Construct
VPVKSEVSLCKDYLRSHLNHVDHKYLLLLDLGFDGTSDRDYEIQTAQLLTGELNFKGARLGDTRKPDVCVYYGEDGLIIDNKAYGKGYSLPIKQADEMYRYIEENKERNEKLNPNKWWEIFDKDVIHYHFAFVSGAFTGGFRERLENIRMRSGIYGAAVNSMNLLLMAEELKSGRLGYKECFKIFDCNDEIVLQRS

SEQ ID NO: 137 - protein, 197 aa, synthetic construct
  REGION 1..197: note = Synthetic Construct
NVLKDKHLEKIKEKFLENTSLDPRFISLIEISRDKKQNRAFEIITAELFNTSYNLSAIHLGGGRRPDVLVYNDNFGIIVDTKAYKDGYGRNVNQEDEMVRYITENNIRKQDISKNNWWKYFSKSIPSTSYYHLWISSEFVGMFSDQLRETSSRTGENGGAINVEQLLIGANQVLNNVLDPNRLPEYMKNQEIIFGTL

SEQ ID NO: 138 - protein, 195 aa, synthetic construct
  REGION 1..195: note = Synthetic Construct
EAIISERATQKERLMQSTDLPMRFYELIDIAYDGRRNRDFEMLTMDLLREGYGFETQLLGGGRKPDVIAYNDDFGIIVDTKAYGKGYHRSQPEEDKMVRYVEDNRERDASVNNTQWWLGFPETLSYQSVYFLWVSSFFTGQFGSQLTNTAIRSRTNGAALGVENLLVGADKFLKGKLNHNQIQLKIRQDSEIIWD

SEQ ID NO: 139 - protein, 196 aa, synthetic construct
  REGION 1..196: note = Synthetic Construct
VPVKSEVSLCKDYLRSHLIHVDHRYLILLDLGFDGTSDRDYEIQTAQLLTAELDFKGARLGDTRKPDVCVYYGEDGLIIDNKAYGKGYSLPIKQADEMYRYIEENKERNEKLNPNKWWEIFDKGVIRYHFAFVSGAFTGGFRERLENIRMRSGIRGAAVNSMNLLLMAEELKSKRLDYNECFKLFDCNDEIGFQRS

SEQ ID NO: 140 - protein, 194 aa, synthetic construct
  REGION 1..194: note = Synthetic Construct
TEADLDSERIKNHYRKITNLPEKYIELLDIAFDHHRHQDFEIITAGLFKECYGLSSIHLGGQNKPDGVVFNSNFGIILDTKAYEKGYGMHINQIDEMCRYIEDNKQRDRIRQPNEWWNNFDDNIPENKFYYLWVSGKFLPKFNEQLKQTHYRTGSNGGGLEVSQLLLGADAVMKGALNVNNLPTYMHNNVIQLV

SEQ ID NO: 141 - protein, 193 aa, synthetic construct
  REGION 1..193: note = Synthetic Construct
NEEKDTLKVKEFFISETSIPNKFITLLDLAYDGNSNRDFEIITSEFIREVYKLNTKHLGGTRKPDILIWNEKFGIIADTKAYSKGYKKNISEEDKMVRYIDENTKRSKEDNPNEWWINFGENIPSNNYFYLWISSEFIGKFEEQLKETASRTNTNGASLNVYQLLMGGHLAQIGRFNVNNLPAFMNNSEIKFS

SEQ ID NO: 142 - protein, 198 aa, synthetic construct
  REGION 1..198: note = Synthetic Construct
NLNLATDEKERLELKEYFISNTNIPSKFITLLDLAYDGKANRDFEIVTAELFEDVFKLKAKHMGGTRKPDILIWTDKFGIIADTKAYSKGYKKNISEADKMVRYVNENNIRNKKDNGNEWWNSFDSNIPEDKYFYLWISSEFVGKFDEQLTETASRTGRDGAAINVYQLLRGADLAQKSQFDVHDFPSLMKNNEIKFV

SEQ ID NO: 143 - protein, 196 aa, synthetic construct
  REGION 1..196: note = Synthetic Construct
VPVKSEVSLCKDYLRSHLAHVDHKYLILLDLGFDGTSDRDYEIQTAQLLTAELDFKGARLGDTRKPDVCVYYGEDGLIIDNKAYGKGYSLPIKQADEIYRYIEENKKRDEKLNPNKWWEIFDKGVVRYHFAFVSGAFTGGFKERLDNIRMRSGICGAAINSMNLLLMAEELKSGRLGYEECFALFDCNDEITFQSF

SEQ ID NO: 144 - protein, 198 aa, synthetic construct
  REGION 1..198: note = Synthetic Construct
NLKLTVDEKERLELKEYFISNTRIPSKYITLLDLAYDGNANRDFEIVTAELFKDIFKLQSKHMGGTRKPDILIWTDKFGVIADTKAYSKGYKKNISEADKMVRYVNENTNRNKVDNTNEWWNSFDSRIPKDAYYFLWISSEFVGKFDEQLTETSSRTGRNGASINVYQLLRGADLVQKSKFNIHDLPNLMQNNEIKFI

SEQ ID NO: 145 - protein, 197 aa, synthetic construct
  REGION 1..197: note = Synthetic Construct
NVLKDKHLEKIKEKFLENTSLDPRFISLIEISRDKKQNRAFEIITAELFNTSYNLSAIHLGGGRRPDVLAYNDNFGIIVDTKAYKNGYGRNVNQEDEMVRYITENKIRKQDISKNNWWKYFSKSIPSTSYYHLWISSEFVGMFSDQLRETSSRTGENGGAMNVEQLLIGANQVLNNVLDPNRLPEYMENKEIIFGTL

SEQ ID NO: 146 - protein, 193 aa, synthetic construct
  REGION 1..193: note = Synthetic Construct
NGEKDTLKVKEFFISETSIPNKFITLLDLAYDGNSNRDFEIITSEFIREVYKLNTKHLGGTRKPDILIWNEKFGIIADTKAYSKGYKKNISEEDKMVRYIDENTKRSKEDNPNEWWINFGENIPSNNYFYLWISSEFIGKFGEQLKETASRTNTNGASLNVYQLLMGGHLAQIGRFNVNNLPAFMNNSEIKFS

SEQ ID NO: 147 - protein, 198 aa, synthetic construct
  REGION 1..198: note = Synthetic Construct
NLKLTSREKSRLNLKEYFVSNTNLPNKFITLLDLAYDGKANRDFELITSELFREIYKLNTRHLGGTRKPDILIWNENFGIIADTKAYSKGYKKNISEEDKMVRYIDENIKRSKDYNPNEWWKVFDNEISSNNYFYLWISSEFIGKFEEQLQETAQRTNVKGASINVYQLLMGAHKVQTKELNVNSIPKYMNNTEIKFL

SEQ ID NO: 148 - protein, 202 aa, synthetic construct
  REGION 1..202: note = Synthetic Construct
TPAESDISSEKLKNHFRRITDLPEKYINLLDIAFDKDRNRDFEIITASLFKEGYGLSSIHLGGQNKPDGVIYNDNFGIILDTKAYGKGYGKYISQIDEMVRYIQDNQERDTFRNPNRWWENFSEFIPKDSYYYLWVSGKFLPTFTEQLKQTNHRSHVNGGGLEVQQLLLGADAVMKGNLDVNDLPKYMKNEVIRFSSSESKI

SEQ ID NO: 149 - protein, 204 aa, synthetic construct
  REGION 1..204: note = Synthetic Construct
PVLKDAALQKTKNTLLNELTEIDPADIEVIEMSWKKATTRSQNTLEATLFEVKVVEIFKKYFELNGEHLGGQNRPDGAVYYNSTYGIILDTKAYSNGYNIPVDQQREMVDYITDVIDKNQNVTPNRWWEAFPATLLKNNIYYLWVAGGFTGKYLDQLTRTHNQTNMDGGAMTTEVLLRLANKVSSGNLKTTDIPKLMTNKLILS

SEQ ID NO: 150 - protein, 200 aa, synthetic construct
  REGION 1..200: note = Synthetic Construct
EIQDQRIAAKKAQFLENTNINPKYLELLDIAYNGSRNRDFEILTADLFNNVFGVDTILLGGGRKPDAIINDNNFGVIIDTKAYESGYSKNITEEDKMVRYIEDNQYRDTERNSTAWWGDFKDTIPTTEFYFMWVSSKFIGEFHTQLEATNKRTQTNGCSINVEQLLIGADLVLKNQLHTKNFPEYMQNKEINWRDLGLIH

SEQ ID NO: 151 - protein, 196 aa, synthetic construct
  REGION 1..196: note = Synthetic Construct
AEADLNSEKIKNHYRKITNLPEKYIELLDIAFDHRRHQDFEIVTAGLFKDCYGLSSIHLGGQNKPDGVVFNNKFGIILDTKAYEKGYGMHIGQIDEMCRYIDDNKKRDKVRQPNEWWKNFGDNIPKDQFYYLWISGKFLPRFNEQLKQTHYRTSINGGGLEVSQLLLGANAAMKGKLDVNTLPEHMNNQVIKLVHQ

SEQ ID NO: 152 - protein, 195 aa, synthetic construct
  REGION 1..195: note = Synthetic Construct
ANADIYLENMKNHYRKITNLPERYLELLDVAFDHNRHQDFEIMTAGIFKDCYGLSSIHLGGQNKPDGVIYNNNFGIILDTKAYEKGYGMHIDQIDEMCRYIYDNKQRDIVRQPNEWWNNFDKNIPKDQFYYLWVSGKFLKNFDKQLKNTHYRTNINGGGLEVSQLLLGADAVMKGNLDVNTLPNYMKNNVIKLVI

SEQ ID NO: 153 - protein, 196 aa, synthetic construct
  REGION 1..196: note = Synthetic Construct
AEADLNSEKIKNHYRKITNLPEKYIELLDIAFDHRRHQDFEIVTAGLFKDCYGLSSIHLGGQNKPDGVVFNNKFGIILDTKAYEKGYGMHIGQIDEMCRYIDDNKKRDIVRQPNEWWKNFGDNIPKDQFYYLWISGKFLPRFNEQLKQTHYRTSINGGGLEVSQLLLGANAAMKGKLDVNTLPKHMNNQVIKLVHQ

SEQ ID NO: 154 - protein, 193 aa, synthetic construct
  REGION 1..193: note = Synthetic Construct
QESKEHEEIKNTFRRKTNLPEKYLELLDIAFDPKRNRDFEIITTDLFRDVYKLEAVHLGGGSKPDGVVYNNNFGIILDTKAYEKGYGKDIKQIDEMVRYIEDNAERDRKRNPNMWWENFGFDIPGNNYYYLWVSGKFLPRFQEQLKMTNYRTEVNGGGLNVRQLLWGADAVQKGELDVNEIPRYMNNTVIEFV

SEQ ID NO: 155 - protein, 200 aa, synthetic construct
  REGION 1..200: note = Synthetic Construct
RISPSNLEQTKQQLREELIYLDHQYLDILDFSIAGNTGARQFEVRIVELLNEIIIAKHLSGGNRPEIIGFNPRENPEDCIIMDSKAYREGFNIPANERDKMIRYVEEYNAKDNTLNNNKWWKNFESPNYPTNQVKFSFVSSSFIGQFTNQLTYINNRTNVNGSAITAETLLRKVEKVMNVNAEYNLSNFFEELGNNTLVA

SEQ ID NO: 156 - protein, 200 aa, synthetic construct
  REGION 1..200: note = Synthetic Construct
RISPSNLEQTKQQLREELINFDHQYLDILDFSIAGNVGARQFEVRIVELLNEIIIAKHLSGGNRPEIIGFNPKENPEDCIIMDSKAYKEGFNIPANERDKMIRYVEEYNAKDNTLNNNEWWKNFESPNYPTNQVKFSFVSSSFIGQFTNQLTYINNRTNVNGSAITAETLLRKVENVMNVNTEYNLNNFFEELGSNTLVA

SEQ ID NO: 157 - protein, 200 aa, synthetic construct
  REGION 1..200: note = Synthetic Construct
RISPSNLEQTKQQLREELINLDHQYLDILDFSIAGNVGARQFEVRIVELLNEIIIAKHLSGGNRPEIIGFNPKENPEDCIIMDSKAYKEGFNIPANERDKMIRYVEEYNAKDNTLNNNKWWKNFESPNYPTNQVKFSFVSSSFIGQFTNQLTYINNRTNVNGSAITAETLLRKVENVMNVNTEYNLNNFFEELGSNTLVA

SEQ ID NO: 158 - protein, 197 aa, synthetic construct
  REGION 1..197: note = Synthetic Construct
KQIKDKYLEDLKLELYKKTNLPNKYYEMVDIAYDGKRNREFEIYTSDLMQEIYGFKTTLLGGTRKPDVVSYSDAHGYIIDTKAYANGYRKEIKQEDEMVRYIEDNQLKDVLRNPNKWWECFDDAEHKKEYYFLWISSKFVGEFSSQLQDTSRRTGIKGGAVNIVQLLLGAHLVYSGEISKDQFAAYMNNTEINFEGA

SEQ ID NO: 159 - protein, 200 aa, synthetic construct
  REGION 1..200: note = Synthetic Construct
NLTPSSLEQTKQVLRTELNTLDHKYLDLLDFSISGTSGARQFEVRIVELLNEIIIAKHLSGGNRPEIIGFNPKENPLDCLIFDSKAYSKGFNIPANERDKMIRYIEEYNVKNETLNSNKWWEEFKSPNYPTNEVKFGFVSSSFNGQYLSQLAYITNRTNRNGCLMSVETLLKKVYNILNTNNKYDLTSFFAEIGSNQFLN

SEQ ID NO: 160 - protein, 201 aa, synthetic construct
  REGION 1..201: note = Synthetic Construct
SISKTDITQLKEKIRENLKTVDHKYLVLVDLAYSDASTKGKKNADAREFEIQTAELFTRELNFSGMRLGDANRPDVIISYEDFGAIIDNKSYKDGFNIDRKCADEMSRYINENTRRVPGIPKNEWWKNFDIKVHTFYFLFITSFLKGNFKSQLDYISKSQSDIQGGAVSVDNLLYIAEKLKSGVIRYEDFFKLFVNEDIIV

SEQ ID NO: 161 - protein, 201 aa, synthetic construct
  REGION 1..201: note = Synthetic Construct
SISKTDITQLKEKIRENLKTVDHKYLVLVDLAYSDASTKGKKNADAREFEIQTAELFTRELNFSGMRLGDANRPDVIISYEDFGAIIDNKSYKDGFNIDRKCADEMSRYINENTRRVPGIPKNEWWKNFDIKVHTFYFLFITSFLKGNFKSQLDYISKSQSDIQGGAVSVDNLLYIAEKLKSGVIRYEDFFKLFANEDIIV

SEQ ID NO: 162 - protein, 195 aa, synthetic construct
  REGION 1..195: note = Synthetic Construct
EEISDIALQKEKAYFYKNTALSKRHISILEIAFDGSKNRDLEILSAEVFKDYYQLESIHLGGGLKPDGIAFNQNFGIIVDTKAYKGAYSRSRAEADKMFRYIEDNKKRDPKRNQSLWWRSFNEHIPANNFYFLWISGKFQRNFDTQINQLNYETGYRGGALSARQFLIGADAIQKGKININDLPSYFNNSVISFE

SEQ ID NO: 163 - protein, 209 aa, synthetic construct
  REGION 1..209: note = Synthetic Construct
IPVKENHTFQTTEADNLKRKLLPVLKHVDHKYLQAIDIAYKKNTSNAENTLLEVLSTDLFVKEMDYKGSHLGGSNKPDAFVYTSKAGWILDSKAYSDGFHVTAANTDAMGRYIQQYRDHKDKSTWWKKFPNNLPITYFAYISSFYNGNYQSQLKDFEDRNKMRGGLIEIPKLILLAEEYQDKKISQAQINQQLLDDKIDWKDYSTILLP

SEQ ID NO: 164 - protein, 195 aa, synthetic construct
  REGION 1..195: note = Synthetic Construct
EEISDIALQKEKAYFYKNTALSKRHISILEIAFDGSKNRDLEILSAEVFKNYYQLESIHLGGGLKPDGIAFNQNFGIIVDTKAYKGAYSRSRAEADKMFRYIEDNKKRDPKRNQSLWWRSFNEHIPANNFYFLWISGKFQRNFDTQINQLNYDTGYRGGALSARQFLIGADAIQKGKININDLLSYFNNSVISFE

SEQ ID NO: 165 - protein, 195 aa, synthetic construct
  REGION 1..195: note = Synthetic Construct
EEISDIALQKEKAYFYKNTALSKRHISILEIAFDGSKNRDLEILSAEVFKDYYQLESIHLGGGLKPDGIAFNQNFGIIVDTKAYKGVYSRSRAEADKMFRYIEDNKKRDPKRNQSLWWRSFNEHIPANNFYFLWISGKFQRNFDTQINQLNYETGYRGGALSARQFLIGADAIQKGKIDINDLPSYFNNSVISFE

SEQ ID NO: 166 - protein, 209 aa, synthetic construct
  REGION 1..209: note = Synthetic Construct
LPKKDNVQRQQDELRPLLKHVDHRYLQLVELALDSSQNSEYSMLESMTMELLLTHLDFDGASLGGASKPDGIAWDKDGNFLIVDTKAYDNGYSLAGNTDKVARYIDDVRAKDPNRASTWWTQVPESLNVDDNLSFMYVSGSFTGNYQRLLKDLRARTNARGGLTTVEKLLLTSEAYLAKSGYGHTQLLNDWTDDNIDHSEYYDKIVNQI

SEQ ID NO: 167 - protein, 195 aa, synthetic construct
  REGION 1..195: note = Synthetic Construct
EEISDIALQKEKAYFYKNTALSKRHISILEIAFDGSKNRDLEILSAEVFKNYYQLESIHLGGGLKPDGIAFNQNFGIIVDTKAYKGAYSRSRAEADKMFRYIEDNKKRDPKRNQSLWWRSFNEHIPANNFYFLWISGKFQRNCDTQINQLNYDTGYRGGALSARQFLIGADAIQKGKININDLPSYFNNSVISFE

SEQ ID NO: 168 - protein, 202 aa, synthetic construct
  REGION 1..202: note = Synthetic Construct
TFKASEADKIKEKLLPVLHNLDHTYLQAVDIAYKDKTTNQENAQLEILSTSLFTKEMEFRGLHLGGVNKPDGFAYDDNDGWIIDSKAYHNGFPLTVSHTDAMGRYIRQYRDRNDNSNWWKTLPSNLPNTQFIYVSSFFIGNYKKQLKDFETRNKMKGSLMEIPQLILLAERYKAGKSSHEEFKNYALANKHNFNEYLAELTK

SEQ ID NO: 169 - protein, 203 aa, synthetic construct
  REGION 1..203: note = Synthetic Construct
ACVKENINDLKDKIRGKLKTLDHKYLVLIDLAYSDASSKTKKNADAREFEIQTADLFTGELAFSGMRLGDSNKPDVIISHGDKGTIIDNKSYQDGFNISAGCRDEMSRYIKENIMRSPALNPNKWWENFDPKVTDYTFLFITSYLKGQFANQLEYISVAHGGIKGAAISVENLLYLSEGIKSGKIRHEDFYNSFHNKEMIFTL

SEQ ID NO: 170 - protein, 203 aa, synthetic construct
  REGION 1..203: note = Synthetic Construct
ACVKENVNDLKDKIRGKLKTLDHKYLVLIDLAYSDASSKTKKNADAREFEIQTADLFTGELSFSGMRLGDSNKPDVIISYGDKGTIIDNKSYQDGFNISAGCRDEMSRYIKENIMRSPTLNPNKWWENFDPKITDYTFLFITSYLKGQFANQLEYISVAHGGIKGAAISVENLLYLSEGIKSGKISHEDFYNSFHNKEMIFTL

SEQ ID NO: 171 - protein, 206 aa, synthetic construct
  REGION 1..206: note = Synthetic Construct
TLQKSDIEKFKNQLRTELTNIDHSYLKGIDIASKKTTTNVENTEFEAISTKVFTDELGFFGEHLGGSNKPDGLIWDNDCAIILDSKAYSEGFPLTASHTDAMGRYLRQFKERKEEIKPTWWDIAPDNLANTYFAYVSGSFSGNYKAQLQKFRQDTNHMGGALEFVKLLLLANNYKAHKMSINEVKESILDYNISYEEYAPLLTEIE

SEQ ID NO: 172 - protein, 195 aa, synthetic construct
  REGION 1..195: note = Synthetic Construct
EEISDIVLQKEKAYFYKNTALSKRHISILEIAFDGSKNRDLEILSAEVFKDYYQLESIHLGGGLKPDGIAFNQNFDIIVDTKAYKGVYSRSRAEADKMFRYIEDNKKRDPKRNQSLWWRSFNEHIPANNFYFLWISGKFQRNFDTQINQLNYETGYRGGALSARQFLIGADAIQKGKIDINDLPSYFNNSVISFE

SEQ ID NO: 173 - protein, 206 aa, synthetic construct
  REGION 1..206: note = Synthetic Construct
VLEKSDIEKFKNQLRTELTNIDHSYLKGIDIASKKKTSNVENTEFEAISTKIFTDELGFSGKHLGGSNKPDGLLWDDDCAIILDSKAYSEGFPLTASHTDAMGRYLRQFTERKEEIKPTWWDIAPEHLDNTYFAYVSGSFSGNYKEQLQKFRQDTNHLGGALEFVKLLLLANNYKTQKMSKKEVKKSILDYNISYEEYAPLLAEIE

SEQ ID NO: 174 - protein, 209 aa, synthetic construct
  REGION 1..209: note = Synthetic Construct
LPKKDNVQRQQDELRPLLAHVDHRYLQLVELALDSSQNSEYSMLESMTMELLLTYLDFDGASLGGANKPDGIAWDSDGNFLIVDTKAYDNGYSLAGNTDKVARYIDDVRARDSNRTSTWWTQVPESLNVDDNLSFMYVSGSFTGNYRKLLKDLRARTNARGGLTTVEKLLLTSEVYLTNNKYGHTQLLRDWTNDAIEHDEYYDQLVANI

SEQ ID NO: 175 - protein, 210 aa, synthetic construct
  REGION 1..210: note = Synthetic Construct
LPHKDNVIKQQDELRPMLKHVNHKYLQLVELAFESSRNSEYSQFETLTMELVLKYLDFSGKSLGGANKPDGIAWDPLGNFLIFDTKAYKHGYTLSNNTDRVARYINDVRDKDIQRISRWWQSIPTYIDVKNKLQFVYISGSFTGHYLRLLNDLRSRTRAKGGLVTVEKLLLTTERYLAEADYTHKELFDDWMDDNIEHEEYFYSLQDALK

SEQ ID NO: 176 - protein, 206 aa, synthetic construct
  REGION 1..206: note = Synthetic Construct
TFSPDAAQVAKEKLRPLLQNVSHSYLYAIDLAFKDKTTAKENAELEIISTQAFDYFNYETKHLGGQRRPDGIATSSEENWVIDTKAYHNGFSLTVNHTDAMVRYMRQADGQIQSDDANELWWRDLTPDVPARYIYISSKFIGNYEAQNRSLMNVTGHEGSVAPVAKLLLLAELKLRDKLTKEQFIQELLSPTGSFEEYLPTFESML

SEQ ID NO: 177 - protein, 202 aa, synthetic construct
  REGION 1..202: note = Synthetic Construct
ETFDSTVADNLKNLILPKLKELDHKYLQAIDIAYKRSNTTNHENTLLEVLSADLFTKEMDYHGKHLGGANKPDGFVYDEETGWILDSKAYRDGFAVTAHTTDAMGRYIDQYRDRDDKSTWWEDFPKDLPQTYFAYVSGFYIGKYQEQLQDFENRKHMKGGLIEVAKLILLAEKYKENKITHDQITLQILNDHISQDEYIKDF

SEQ ID NO: 178 - protein, 204 aa, synthetic construct
  REGION 1..204: note = Synthetic Construct
TRLAADPVKVRDVLRQRFSAGYGGFLMHYTELAQGSNTAATKFEQATTEIFSKVFGYRAKHIGAQPLRPDVVLYSETDRYGAILDTKAYAKRYTLSHDQRGVMRNYVVDYPKYKIGDGDLAFFSYVSGRFGPNIDAQLAEVSERADGVPGSAITAHDIVLMCKRHLGAEKYTHAQLREFFSGNKQVQVAGHERSLADLVAAATA

SEQ ID NO: 179 - protein, 191 aa, synthetic construct
  REGION 1..191: note = Synthetic Construct
GLERAMVARVAQQVLGRDRTVDQFLSTYANLVHDESPRAAKLFEESTANILKAVFRVDAKLVGSQGREPDVVVSGDGWRGIVDTKAYSGEYTLPSGHDRAMREYVENYRAGDSPLRFWAFICGAVARGASAKVHFLGKQVGLAGTVVGMVAWLQMIKLAEAGVIGGSDLPRLFSIGRELTLEDLPTLVAGG

SEQ ID NO: 180 - protein, 199 aa, synthetic construct
  REGION 1..199: note = Synthetic Construct
GFSHSEVEKAAKKVLGTDRTLDNFLYSYQSLPYSSAKDAPRKFELATAELFRRVFKLDAECVGQAGREPDVVVTKPGEWRGIVDTKAYSGDYSLPSSHERAMREYVETYRAAPGAPLRFWVFIAASVSKGARHRVRQLADLVDSPGAVIGMLAWTEMIRFAQKGKIDSERMADLFALNSELTMEDLKKVLSADRDVSLG

SEQ ID NO: 181 - protein, 212 aa, synthetic construct
  REGION 1..212: note = Synthetic Construct
LLVDGATSDIISRLVAETGYEYSEVEVAAKKVLGTDRTLDSFLSNYQSLVFSDDKSAPRYFERATAEIFRRIFNLEAECVGQSGREPDVVVTKRDAWRGIVDTKAYSGEYSLPSEHERAMREYVETYRAVPGAPLSFWVFIAGSISKGAKHRVRGLADRVDSPGSVIGMLAWTEMIRLAQDGKIDADRMAELFKSNSELTLDDVRRLPKADV

SEQ ID NO: 182 - protein, 203 aa, synthetic construct
  REGION 1..203: note = Synthetic Construct
SGYLDLEEASRAAFFNDDGIHWFITGDIAEIHSDGTFSIIDRKKDIVKLANGEFISLGKIEATLKSSCYVDNICIVPNATLNCLVALIVPNLMSIKSLIGRQLELTKQLPQLSDPNLLIGHPEIIKIIHNDIIDVGIRQRLKSLELPSMITLCEEIWAPDNDLLTAAMKLKRANIIKHYNYDLQQMWSSLRANPEKIRLQLKK

SEQ ID NO: 183 - protein, 205 aa, synthetic construct
  REGION 1..205: note = Synthetic Construct
QFSHGEVEKVARRILGTDRTLSSYLLHYQSLVTSSDRNAPREFEQATAEIIRRVFKLEATCVGQTGREPDIVVRKPGEWRGIIDTKAYGGEYSLPSGHDRAMREYVEKYSGDGGDDLRFWVFLAGSLSKNAGARARELAQRIGCQGVVIGLSAWMKMIELGQAGKLSGDKLGWLFSLDGELTHADIARAQEAASFAELHAQRGLF

SEQ ID NO: 184 - protein, 199 aa, synthetic construct
  REGION 1..199: note = Synthetic Construct
PERQRTIHDKRKEKIMERTSLPLKFYELYDIAFDPKRSRDFEILTVELFKLATNTNARVLGGSLRPDGIVYQQADGQSPGIIIDTKAYADGYSKIKSQEDEMVRYIEDNQFRDPKRNPTKWWESFPKTISPKNTTFLWVSSTFTGAFDEQLKSTYHRTNANGGAVAVDQLLIGVDKVCRGELTSEELFDSLKRNQIATF

SEQ ID NO: 185 - protein, 193 aa, synthetic construct
  REGION 1..193: note = Synthetic Construct
SKEKSNLKLKEFFISETAIPNKFITLFDLAYDGSANRDFEIITSELFRDVYKLNTKHLGGTRKPDILIWNKEYGIIADTKAYSKGYKKNISEEDKMVRYIDENIKRNKNDNPNEWWKIFDKSISSANYFYLWISSEFVGKFEEQLQGTATRTNTNGASLNVYQLLMGAHLVQIEELSVNSIPAYMNNMEIKFV

SEQ ID NO: 186 - protein, 198 aa, synthetic construct
  REGION 1..198: note = Synthetic Construct
TRRRDEIEERIVRLGARLRHVPDRYLDLVRLGFDPSRSADFEFGVFEVFRDLLGYDALKLGGGLAPDALAWYADPQFLPLSYGLIIDAKSSATAFSVDVSAADQMTRYVLEYQKELLSRHIPTAYFLFVGGAFSGPLGGLRLLHERTRVAGAAITIADLIHLAEQLRERRQEVTLRSVSALFGSLQLIDAAKIDALHG

SEQ ID NO: 187 - protein, 194 aa, synthetic construct
  REGION 1..194: note = Synthetic Construct
PVARVDWVLAQKYPSGAVDGFMNSYAQMAFESREKATDFEKATTSIFRDVFGFEARHIGAYSERPDVVISSHEAGYGAILDSKAYKKGYSLGVSQRNRMRDYISNFEEYALDSNPLAFFAYVVSEYKSNVESQLRDVAEENGVNGAAITARDIIRMVRRHRDRPYSHEEIRAIFSGNRPVVLSDLQDLSEGAFR

SEQ ID NO: 188 - protein, 201 aa, synthetic construct
  REGION 1..201: note = Synthetic Construct
GIDRSTVSSVLQMKFPRGASEAFLSNYLELSARSREKATEFEVATAEIFRKIFGFKAEHTGNHGLRPDVVLSSTEAHYGAIIDNKAYKKGYSLGVSQQGRMRDYIEDFPRYRLSEDEERPAFFVYVIHEGSTNLTSQIQALSEKTGVHGSAITARDILLMVRRHQEKPFTHEEIRSLFSQNQIVDLLDDGYEGLGDRVLGA

SEQ ID NO: 189 - protein, 194 aa, synthetic construct
  REGION 1..194: note = Synthetic Construct
ASTGFSPASVSAALGRVMPDRSRTLDQFLLGYAEMARSSRERARDFELATTDVFKRVFELDARHVGGAGREPDVVVDNNNSWRIIVDTKAHGNGYTLPASDERAMKEYVAAYAQKSPKLKAWVFISSSFGASINPRLRKIVDETGVPGSAVGITAWIALIQHAQDGRVDAEMLLALLSVGREVTLEDVQRVVVG

SEQ ID NO: 190 - protein, 191 aa, synthetic construct
  REGION 1..191: note = Synthetic Construct
REISLATGLTVSAVESGLSGWSADTLGIFEASYVDMAFSSREKALDFELATVDLFKQLGFSTRHVGASPRHPDVLIESPLCYSGIIDNKAYSAYSISNDHRNRMEQNYIPTYQSSHGDLAFFMYIAGGFINTIDNQIARIAMTSGVAGSAIKASDMIKILQKHQNSVIDHNLLKALFRANRRITIQDIHSL

SEQ ID NO: 191 - protein, 185 aa, synthetic construct
  REGION 1..185: note = Synthetic Construct
SGFDEKIVEETLLRLYPNGAVGSFMTEYFELAFKGRDNAIEFEKATVELFKNIFGFETKHIGSVGLNPDVYVLSNEGKYIGILDNKAYRRYTISNDHRNRMVHNYIEQYKSDVYPLAFFSYISGGFGSNIDSQIKSISDETQVNGSAMSVTNMIRMVEKHAQKQYSHSSIKDIFSLNRQVVLSDL

SEQ ID NO: 192 - protein, 202 aa, synthetic construct
  REGION 1..202: note = Synthetic Construct
ERIKKEIQKTITYVVGKTQNLDENLIEKVIEQSFSGKKSCKEFEDSIFKLYSETIGFEGIKLGGIGNREPDSLFWYKVHNDEDNYGLIVDAKAYSKGFKINTSSSRQMNDYIYKFYNKLQEEHGLNRSHYHWVTSKYIGNGDIEYFAENVRNMYSFESKGSIISISNALLIADKIQSNRDFKKLESLMSIEREILETDIEVF

SEQ ID NO: 193 - protein, 188 aa, synthetic construct
  REGION 1..188: note = Synthetic Construct
RLVENTLIEAYPNGAISGFMTEYFEMAFKGTEEAIQFEEATTELFSEVFGFKAKHLGQTGSKSAPDVLLLSDDAGYQAIIDNKAYSRYSISGDHHNRMVHNYLNNISNYSEYQQPIGFFTYISGGFGNQIDRQIQSIAEESGIHGSGMSVSNMIKLVEKQNEKPLTHQMIREIFSVDRQILLSDLNLV

SEQ ID NO: 194 - protein, 203 aa, synthetic construct
  REGION 1..203: note = Synthetic Construct
KEIQKEIQKMVDDLKKLSLSIDDGFMEKIITEAYSGRDKCKEFEDSVFELYRDSIGFDGIKLGTIGSREPDSLFWYKVEDTQDSYGLIVDAKAYSKGFKINTNSSRQMNDYIYSFTKKLEADQGVSRSHFHWVTSKYIGKNDIEDFSENVRNMYDFTSLGSIVGVGNALIMADEMKKKKDFTKLENVLTTGREITVEDIRKIS

SEQ ID NO: 195 - protein, 194 aa, synthetic construct
  REGION 1..194: note = Synthetic Construct
ICSKTGIAEQTVERFLLSQYPHGNIDDFFVSYREFANMGRAFAREFEKATCEMFRKIFKMRAEHVGPIGNTPDVLILSESENFCGIIDNKAYHKGYSISGDHKRVMEDVYIPNYQAYGSTKLPLAFFAYIAGSFKKTVNSQLQEITRDTGISGSAMPVDVFINFAQDYANGSCTHRTIKDLFSLNREISLSDLP

SEQ ID NO: 196 - protein, 184 aa, synthetic construct
  REGION 1..184: note = Synthetic Construct
QYSVVEDCLFKIYPHGAIRIFMNEYFEMAFKGRDEATAFEKATSEIFRNVFLFQSEHIGQKGLTPDVVVISDEFGFSGIIDNKAYSKYSINNDHKNRMIHNYIPKYKNFKKCDLAFFMYIAGGFSNSFEISIKNISRESKVNGSGISVVNLIKMIEKQIEKPYCHLSLRSIFSLNRLITPEDMM

SEQ ID NO: 197 - protein, 181 aa, synthetic construct
  REGION 1..181: note = Synthetic Construct
QLVEETLLRLYPRGAIGSFMTEYFDMAFRGRDDATEFELATVELFKNAFDLRAEHIGPQGLTPDVLVLSDQEGFIGIIDNKAYSKYTISNDHRNRMVHNYIPRYRSGQQYPLAFFSYISGGFGSSINAQIKSIVDETHIHGSAISVSNVITLVDLYSQRGYNHARLKDILSLDRQVLLADL

SEQ ID NO: 198 - protein, 197 aa, synthetic construct
  REGION 1..197: note = Synthetic Construct
GISMSKIRAILQKVSKTKPSNDEIALRYLELARGGREAAVAFEQATAEIFGPWGLGFESEWIGAHPNHPDVRVLNVAQAPYYAGILDAKAYEGGYDLPRDHERRMYDEYIPAHRHMKRDEHIVPLRWFGYVSSSFGANFDRKLTRIAQRGGVSGFAISADTLLALVQRHKQRPLTEDEFCDLFSVNREVMVDDFSTA

SEQ ID NO: 199 - protein, 193 aa, synthetic construct
  REGION 1..193: note = Synthetic Construct
LVTETQFEHQEVETAAKQILGTDRTLETYLYNYQALVYSQKRDAPRVFEQATAEILRQVFGLEAVCVGQSGREPDVVVTQPNEWRGIIDTKAYSGEYTLPSSHDRAMREYVERYSATPGETLRFWAFIAGAISRGAGAKATSLSSQTGIPGVVVGMLAWLQLIRLGQEKRVDGEQLADYLSKGGELTVADLSQ

SEQ ID NO: 200 - protein, 184 aa, synthetic construct
  REGION 1..184: note = Synthetic Construct
IPSKYIEEQLDSFRIDTFSLFETNYIDMAFSGREFASEFEHTTMDVFSELGFQTQHVGTKSRQPDIFIQSHDASFSGIIDNKAYHVFSITHDYELKMINSYIPKYKKRYSDFSFFMYIAGGFGKNFDKQVQTIANQSGINGCGIRASDLMRLLKKHKQNPIDHQKLKQIFECNRLVRIQDILSL

SEQ ID NO: 201 - protein, 187 aa, synthetic construct
  REGION 1..187: note = Synthetic Construct
VSLKDTERILSAKYPKGLVDSFLSEYVQMAFESRDKATEFEKATTSIFADIFGLYAEHIGQKGIVPDVVIASREEGWSGILDSKAYAKGYSIGHDHRNRMVEYIERYPEYGPDFAALAFFSYVVSDYKNSVTPQIRLISEKSGVPGSVITARDIVRMVERHKKKPYTHAEIREIFSLNRAITFEDIG

SEQ ID NO: 202 - protein, 189 aa, synthetic construct
  REGION 1..189: note = Synthetic Construct
TGVSAVETERILSAKYPNGLVDSFLSEYVQMAFESRDKATEFEKATTSIFADIFGLYAEHIGQKGIVPDVVVASREEGWSGILDSKAYAKGYSIGHDHRNRMVEYIERYPKYGPEFATLAFFSYVVSDYKNSVTPQIRTISEKSGVPGSVITARDIVRMVERHQKKPYTHSEIREIFSLNRAITFEDIE

SEQ ID NO: 203 - protein, 189 aa, synthetic construct
  REGION 1..189: note = Synthetic Construct
TGVSAVETERILSAKYPNGFVDSFLSEYVQMAFESRDRATEFEKATTSIFADIFGLYAEHIGQKGIVPDVVVASREEGWSGILDSKAYAKGYSIGHDHRNRMVEYIERYPKYGPEFATLAFFSYVVSDYKNSVTPQIRTISEKSGVPGSVITARDIVRMVERHQKKPYAHSEIREIFSLNRAITFEDIG

SEQ ID NO: 204 - protein, 219 aa, synthetic construct
  REGION 1..219: note = Synthetic Construct
TGVDEKTVERFLIQNYPHGNIDDFFLCYKELAHMGTAGARDFETATCEMFRKIFRMRAEHVGPIGNTPDVFVESTDAGYCGIIDNKAYKNGYSISGDHKRVMEDVYIPNYKTYGQTEQPLAFFTYIAGSFGSNINSQLATITRDTGVSGSAMPVDIFINLAQDYADKGYDHKFLKDIFSVNREIQLSDLQPKSKAFQYDFQSQSLGMVAEPTVPYGKKD

SEQ ID NO: 205 - protein, 195 aa, synthetic construct
  REGION 1..195: note = Synthetic Construct
DFDHSEVAKIATNVLGTDRTLDNFLYTYQSLPHSSAKDAPRKFEQATAEIFRRVFKLDAECVGQAGREPDVVVTKPGEWRGIVDTKAYDGDYSLPSSHERAMKEYVETYQNRDGEVLEFWVFIAASVSRGAHRKAKMLAERIETSGVVIGMFAWLEMIRKAGSGSMDSDQMAALFQSSGELTMADVRSGEVSSSR

SEQ ID NO: 206 - protein, 198 aa, synthetic construct
  REGION 1..198: note = Synthetic Construct
VAVKTGISPARVEQVLTQKYPGGSAAWFMAKYVQLAFQSREHATQFEVATTSIFRDVFGFQAQHVGPIPRRPDIVIASLEVHYGALLDSKAYKTGYSATIGQQNRMRDYIDDFPDYALSGAPLAFFAYVVSGTKSTLRAQIQDIARQNGVPGAAITAAQLAAMVERHSTTKYTHEQIRQILSVNREVEMADLAIGDGR

SEQ ID NO: 207 - protein, 194 aa, synthetic construct
  REGION 1..194: note = Synthetic Construct
EESETEIEKLIEKLVVQYEDTIPAKLVDGLVRYGYDGSEGINFEITVAQFFRYLGYKTEYFGQGRGRTADVIARYINKIYARSYGIIIDSKATSDKYTFPAGDIRKMKEYIDLHGRELLKDSIPLHAFAFVSSCFCEDVASPLKEISEDTGIKGTAIEVLKLLEFGCLLTKGKLYIENMYPAYITNSTFDVGNL

SEQ ID NO: 208 - protein, 206 aa, synthetic construct
  REGION 1..206: note = Synthetic Construct
AGISAKFVEEILQKKYPHGSIGAFMANYFELAFNGREDCRKFEIATAEIFKNVFGFTSHHIAGGAKEVPDVLLIAENAGYQAIIDTKAYNRYDLGATQRDRMIYHYLQDIQTYSSSTLPVGFFSYIAGGFSNNIASPLCKIVNATGVNGSAMPVAAFIKMAERQGNSPYTKDEICQIFSVNRKIELSDLDICSSLMVAENSIKYGK

SEQ ID NO: 209 - protein, 186 aa, synthetic construct
  REGION 1..186: note = Synthetic Construct
PATTVEKTLAKTYPDGAVGTFMHSYAQMAFESRDRATDFEKATASVFRDVFGFKAEHIGQRGRVPDVVIASDTEHYGALLDSKAYAKGYSIGISQQNRMRDYITDFPTYRLTDAPLAFFAYVVAEYKSTINGQLKEIAETNGVPGSAITARDIIRMVEHHQDTPYTHAQIRELLSVNRAVTYQDLS

SEQ ID NO: 210 - protein, 187 aa, synthetic construct
  REGION 1..187: note = Synthetic Construct
ITGFSNQQVEAVLQGFRPDTLSIFETSYLNMAISGTELAREFELATNHIFELLGFHSRHIGTSPLHPDVFAASTTYNFSGIIDAKAYRTYSLTNDHRNRMINNYIPDWSNRFGNLSFFMYVADGFGANIDNQIQQVSNASGKNGCVISARDLLYLLQKHLASPVDHSRLNNIFQYNRRLTVVDIESL

SEQ ID NO: 211 - protein, 184 aa, synthetic construct
  REGION 1..184: note = Synthetic Construct
ATGYTTNEVARALDGFRPDTFSLFEATYMNMAVSGRELATEFELATQNVFEELGFNAQHVGAKPLHPDIYVESPLNYSGIIDTKAYRRYSITNDHRNRMVRNYIPTYRDDDFTFFMYVADGFGSNISSQIQSIAEETNINGTVITASNIMRLLQRNQVATIDHASLRNLFTSNEVVSISDINSL

SEQ ID NO: 212 - protein, 190 aa, synthetic construct
  REGION 1..190: note = Synthetic Construct
QTGIDEKLVEEVLLRLYPHGAIGSFMTEYFEMSFKGRDEATEFENVTAELFKIVFGFDAKHIGSIGLTPDVLLLSDVEGYAGIIDNKAYSKYTISNDHHNRMVHNYIRNIKNYYSGSYPLAFFSYIAGGFGRNINTQIRNIAKETSVHGSAMSVSNMIKLVEFHSRTPFSHKHLRDIFSVDRLILISDLE

SEQ ID NO: 213 - protein, 185 aa, synthetic construct
  REGION 1..185: note = Synthetic Construct
SLGYTELQVESALEGFPDTFSVFEAGYLNMAISGTELAKEFEIATQNIFQQLGFISEHVGNNPLHPDVFVESSSGYSGIIDNKAYRAYSINNDHRNRMINNYIPLYKDKHDNLEFFMYIADGFGSNIDNQLLQISQRTQVNGCVITARNLIRLLQKHLVNPIEQSVLRDVFKCNSSITIHDIDAI

SEQ ID NO: 214 - protein, 185 aa, synthetic construct
  REGION 1..185: note = Synthetic Construct
STGYSNHQVEDALANFRPDTFSHFEASYLNMALSGTELAADFEIATGGIFEELGFDSEHVGNQPLHPDVFVRSPLNFSGIIDTKAYRQYTISNDHRNRMINNYIPTYQNGNNLEFFMYVADGFGTNIDTQVQDIATRTNVNGSVITAQNMIRLLQRHSSNPLDHNRLRMLFTQNSIIRLSDINSL

SEQ ID NO: 215 - protein, 186 aa, synthetic construct
  REGION 1..186: note = Synthetic Construct
LTGYTVREVEDALDGFRPDTFSQFEASYLNMAISGTELATEFETATQAIFEQLGFRAEHVGNHALHPDVFVESPLNYSGIIDTKAYVRYVINNDHRNRMVNNYIPTYQNQHGNLEFFMYVAHGFGSNIDSQVQSIADRTNVNGSVITARNVIRLLQRNYANPIDHNTLKTLFTKNSRITMADIDSL

SEQ ID NO: 216 - protein, 186 aa, synthetic construct
  REGION 1..186: note = Synthetic Construct
STGYSIREVEDALDGFRPDTFSQFEASYLNMAISGTELATEFEIATRGIFEQLGFHAEHVGNHALHPDIFVESPQNYSGIIDTKAYRTYTINNDHRNRMVNNYIPTYQNQYGNVEFFMYVADGFGSNIASQVQNIADRTNVNGSVITARNVIRLLQRYQATPIDHNSLRILFANNSVITMSEIDSL

SEQ ID NO: 217 - protein, 189 aa, synthetic construct
  REGION 1..189: note = Synthetic Construct
ATGYNVKEVEESLDGFRPDTFSQFEASYLNMAISGTELATEFEIATGEVFKQLGFCTEHVGSRSLHPDLFVESPKKYSGIIDTKAYRRYTISNDHRNRMTNNYIPNYKNISGNLEFFMYVADGFGNNINSQLQNIADHANTNGSVITARNVIRLLQANQATPIDHDRLKMLFTSNSEITTADIDSCRRR

SEQ ID NO: 218 - protein, 191 aa, synthetic construct
  REGION 1..191: note = Synthetic Construct
RTGINSLTVGAVLQKLYPHGAIGSFMNEYFEMAFRGREDATDFERATQTIFQDTFGFEATHIGAAGLTPDVLVLSDSAGYQAIIDNKAYSKYSISNDHRNRMIHNYINGLASYSKSALPLAFFSYIAGGFSPSIDDQLKSIADESGVPGSAMPVSNMIKLINLHSENKFSHEQLKRIFSIGRRIELKDLIH

SEQ ID NO: 219 - protein, 187 aa, synthetic construct
  REGION 1..187: note = Synthetic Construct
VSGYSEKQVEHALENFHPDTYSLFEVTYLKMASSSRELDTEFEKATIDIFTQLGFSAQHVGNKNLHPDGFVESPLNFSGIFDTKAYARYSITNDHHNRMTINYIPTYQQSNPNLSFFLYVAYGFKNTIDGQIQKIKRVNGVNGSAITAKDLLYLLRRHKTKAIDHADLKKLFESNKRITMQEINRLP

SEQ ID NO: 220 - protein, 184 aa, synthetic construct
  REGION 1..184: note = Synthetic Construct
STGITHSIIEEELANFANGALDSFEASYFDMALKGREQCREFEIATVELFDKAFGFDTSHVGDKGKHPDILAVSEQFSGIIDSKAYASYTISNDHKNRMTHNYIPPYRKQYPNLDFFMYIAGGFGRNFDKQVLSVAQESNLNGCGITANNIIKLARNYKINNWTHDNLQQLFTLNKEIKRTDFT

SEQ ID NO: 221 - protein, 194 aa, synthetic construct
  REGION 1..194: note = Synthetic Construct
VTGINGKTVENVLIETYPNGSVGAFMTRYFEMAFKGRDEATEFEKATVELFQDVFGYKAKHVGPIGLTPDVLLLSDSDGYQAIIDNKAYHKYSISNDHYNRMVHNYIENLANYSDSSDRLAFFSYIAGGFGKNIDKQIQSVANATGVNGSAISVTNMIKMVEQHNKVPYSHKKLCEIFSVNRQVLMQDLILREE

SEQ ID NO: 222 - protein, 186 aa, synthetic construct
  REGION 1..186: note = Synthetic Construct
QTGIEVSIVEETLLKLYPYGAIGSFMTEYFEMAFKGRDEATEFEKATVELFKSVFEFEAQHVGPIGLTPDVYILSHESRYVGIIDNKAYSKYTISNDHRNRMVHNYIKTYSAECYPLAFFSYIAGGFGKNITSQIKDIVDETLIHGSAMSVSNMIKMVENHQYKKYSHDEIRNIFSVDRQILLSDL

SEQ ID NO: 223 - protein, 190 aa, synthetic construct
  REGION 1..190: note = Synthetic Construct
VTGIDGKTVEDVLIETYPNGSVGAFMTKYFEMAFKGRDEATEFEKATVELFHDVFGYKTKHVGPIGLTPDVLLLSDSDGYQAILDNKAYHKYTISNDHYNRMVHNYIENLENYSDAENRLAFFSYIAGGFGKNIDKQIQSIVDATGVNGSAISVTNMIKLVEQHNKVPYSHRRLCDIFSVNRQVLMQDLI

SEQ ID NO: 224 - protein, 190 aa, synthetic construct
  REGION 1..190: note = Synthetic Construct
RTGIDGKTVEDILIETYPNGSVGAFMTKYFEMAFKGRDEATEFEKATVELFQDVFGFEAKHVGPIGLTPDVLLLSDESGFQAILDNKAYHKYTINNDHYNRMVHNYIGNIGNYSKSDEPLAFFSYIAGGFGSNIDKQLKNIVDATDVNGSAISVSNVIKMVEQHREKPYTHQRIKDIFSVNRQVLMKDIV

SEQ ID NO: 225 - protein, 190 aa, synthetic construct
  REGION 1..190: note = Synthetic Construct
QTGIDGKLVEEVLVEQYPTGSVGAFMTKYFEMAFKGREEAVDFEKATVELFHDVFGFESKHVGPIGLTPDVLLISDLDGYQAIIDNKAYSKYTISNDHYNRMVHNYIENLANYSESNNNLAFFSYIAGGFGSNIDGQIRNIVNTTGINGSAISVSNVIRMVDIHNSNPFNHQKIKDVFSMNRQVLLKDLT

SEQ ID NO: 226 - protein, 190 aa, synthetic construct
  REGION 1..190: note = Synthetic Construct
RTGIDGKTVEDILIETYPHGSVGAFMTKYFEMAFKGRDEATEFEKATVELFQDVFGFEAKHVGPIGLTPDVLLVSDSEGYQAILDNKAYHKYTINNDHHNRMVHNYIGNIHNYSKSDKPLAFFSYIAGGFGSNIDKQLNNIVEATGVNGSAMSVSNMIKMVEQHECTPYSHQKIRDIFSLNRQVLINDIL

SEQ ID NO: 227 - protein, 189 aa, synthetic construct
  REGION 1..189: note = Synthetic Construct
KTGIDGKFVEETLLKFYPRGAIGSFMTEYFEMAFRGRDEATEFERATTCLFKDVFNFETHHVGPIGLTPDVLLISDQEGYCGIIDNKAYSKYSISNDHHNRMVHNYIEGFSRYCQSQNPLAFFSYIAGGFGNNINGQIQSIVHEAGVHGCAFAVTNVIQLVEKHQVMPYSHLDLKDIFTLDRQVLLSDL

SEQ ID NO: 228 - protein, 190 aa, synthetic construct
  REGION 1..190: note = Synthetic Construct
QTGIDDKTVENILIETYPNGSIGGFMTKYFEMAFKGRDEATEFEKATAELFQDVFGFETKHVGPIGLTPDVLLISDCAGYQAIIDNKAYHKYTINNDHYNRMVHNYIGNMNKYSSSNNALAFFSYIAGGFGSHIDSQIKSIADATGVNGSAMSVTNVIKMVEQHNKQPYSHEKIKDIFSVNRQVLMNDII

SEQ ID NO: 229 - protein, 189 aa, synthetic construct
  REGION 1..189: note = Synthetic Construct
QTGFDDKLVEETLLRLYPRGSVGAFMTEYFEMAFKGRDEATPFEKATVELFQDVFGFEAKHVGPIGLTPDVLLVSDVEGYQAIIDNKAYSKYTISNDHHNRMVHNYIENLGRYSSSAAPLAFFSYIAGGFGKNFDSQVRAIVDETGVNGSGFSVSTMIKLVECYSDKGYTHKTLRDLFSLNRQVLMTDF

SEQ ID NO: 230 - protein, 189 aa, synthetic construct
  REGION 1..189: note = Synthetic Construct
ATGIDGKTVEEVLIETYPRGSIGSFMTKYFEMAFKGRDEATEFEKATVELFRDVFGYQTKHVGPMGLTPDVLLVSPECSYQAIIDNKAYSNYSINNDHRNRMVHNYLTNISRYSDREYPMAFFTYIAGGFGTAIDKQIESIYEESGVRGSAVSVTNIIKMVEKHQESAYTHQDLRNLFGVNRQILMRDL

SEQ ID NO: 231 - protein, 190 aa, synthetic construct
  REGION 1..190: note = Synthetic Construct
VTGIDGKTVENVLVETYPNGSVGAFMTKYFEMAFKGRDEATEFEKATVELFQDVFGFEARHVGSIGLTPDVLVLSDEDGYQAILDNKAYHKYTISNDHFNRMVHNYIGNISSYGDGDKSLAFFSYIAGGFGTNIDKQLKNIVDATGVSGSAVSVSNMIKLVEQHNQTPYSHKRIKEIFSVNRQVLLSDLA

SEQ ID NO: 232 - protein, 187 aa, synthetic construct
  REGION 1..187: note = Synthetic Construct
QTGIEAKIVEDTLQKNYSRGAIGSFMVEYFEMAFKGRDEATEFELATAELFKSAFGLTTEHIGSKSLMPDVLVLSDQFKYIGIIDNKAYSSYSITNDHKNRMMYNYIPAYKKEQKYPLAFFSYIAGGFGTNIDSQIKEIVDSTNINGSAISVSNVINLVTNYQSKGYNHTKIKNIFSIDRQVLISDL

SEQ ID NO: 233 - protein, 187 aa, synthetic construct
  REGION 1..187: note = Synthetic Construct
QTGIDARFVEETLLKYYPHGAIGSFMTEYFEMAFRGRDDATEFELATVELFKSAFGFETEHVGPIGLTPDVLILSNQDNYIGIIDNKAYSKYTISNDHKNRMIHNYIKTYKQEQKYPLAFFSYIAGGFGKNINSQIKEIVDESKINGSAISVTNLIKLVEYYGTKNYDHGKIRDIFSVNRQVLMSDL

SEQ ID NO: 234 - protein, 191 aa, synthetic construct
  REGION 1..191: note = Synthetic Construct
RTGIDPRVVEEILIEKYPHGSPSAFMSEYFSMAFKGREEAADFEKATVELFQNVFGYEASHVGPIGRSPDVLLESKSAHYQAILDNKAYSRYTVSNDHHNRMVDNYIRDKAHYSTSPYPLAFFSYIAGGFGSNIDPQIQSIVHDGGVNGSCITVSNVIQMVENSETKPYTHEKLRQIFGLNRQVLISDLQQ

SEQ ID NO: 235 - protein, 189 aa, synthetic construct
  REGION 1..189: note = Synthetic Construct
KTGCNAKVVEEKLCKLYPNGAVGSFMTEYFNMAFKGTEQAADFEKATVELFRDVFGYETEHVGSIGLTPDVLLVSDSDGYQAIFDNKAYSSYSISNDHRNRMIHNYIENLGKYSKHSHPLAFFSYIAGGFGNKIDSQIQSVVQETGISGSAISVSNVISLVEKHQSNPYSHKQLKDLFSLERQILLSDL

SEQ ID NO: 236 - protein, 189 aa, synthetic construct
  REGION 1..189: note = Synthetic Construct
QTGIDGRLVEENLQRLYPHGAIGAFMTQYFDMATKGRDEATEFEKATVTIFNEVFGFNSKHVGPIGLTPDVLLLSDSDKYSAIIDNKAYSRYSISNDHHNRMIHNYIEGFKNYCDSPYPLAFFSYIAGGFGSNIDAQLMKIVNETGVNGSAVTVSSVIQMVEKQQAEPYSHAKIRELFSLNRQLVLSDL

SEQ ID NO: 237 - protein, 189 aa, synthetic construct
  REGION 1..189: note = Synthetic Construct
KTGFLPDLVEDCLQELYPQGAIGAFLSEYFEMAFKGREQATDFELATVDLFQNVFGFTARHVGPKGLTPDVLLLSDDEGYSAILDNKAYSKYSITNDHHNRMVYNYIGQLNNYYNGTYPLSFFSYIAGGFGSNINIQLNRVVNETGINGSAINISTMINLVYEHTSNPYTQQRIRDIFSLNRRVLQADL

SEQ ID NO: 238 - protein, 186 aa, synthetic construct
  REGION 1..186: note = Synthetic Construct
VSGFEYRVVEQILLRKYPHGAIGSFMSNYFEMAFRGRDEAIEFETATVEIFENVFGMKANHVGPIGLTPDILVISDDAGYLGIIDNKAYSRYSITNDHKNRMIYNYIPSYQRDEYPLAFFTYIAGGFGNNINRQLNDISSATNVHGSAINVSNMIQLVQNFSEYSYDHFTLKDIFSLDRQITQSDI

SEQ ID NO: 239 - protein, 192 aa, synthetic construct
  REGION 1..192: note = Synthetic Construct
DTGIAGNTVEEVLQKNYPHGAIGSFMTEYFEMAFKGRDEATEFEVATRTIFEETFGFKARHVGPIGLTPDVLLLSDNAGYQAIIDNKAYSKYSISNDHRNRMVHNYINGLANYSQSSLPLAFFSYIAGGFSPSIDAQLKSITEETGIKGSAMPVSNMIRLINQHSETPFTHEQLRGIFSLNRKIELKDLIHS

SEQ ID NO: 240 - protein, 181 aa, synthetic construct
  REGION 1..181: note = Synthetic Construct
EQILSKKYPYGFGDLFLQKYIELSRGGRKRATEFEKATSSIFADMFGVCAEHIGQKGSVPDIVVGSRDGKWAGILDTKAYNKKYSISNDHKNRMIGYIERYSEYGFEFANLSFFAYVVSDYGKNINSQIRYISNKSGVLGSAVTARDIIRMVERHQKKPYTHDEIREIFSVNRAITLKDID

SEQ ID NO: 241 - protein, 189 aa, synthetic construct
  REGION 1..189: note = Synthetic Construct
LTGIDSKLVEDTLLRWYPHGAIGSFMTEYQEMAFKGREDATDFEKATVAIFRDSFGFAAEHVGPIGLTPDVLLLSDAAGYQAIIDNKAYSRYSISNDHRNRMVHNYICQLSSYSKSAHPLAFFSYIAGGFGNNISTQIKSIADETGIAGSAVSVFNIIKLAEENQRNPYSHESIRDIFSKNRLIELKDL

SEQ ID NO: 242 - protein, 190 aa, synthetic construct
  REGION 1..190: note = Synthetic Construct
STGLKESFVWEILQKRFPRGSIGAFMTQYYEMAFKGREEATEFEKATAELFHDVFKFKTKHVGPIGLTPDVLIESEDVGFVGIIDNKAYSKYSISNDHHNRMVHNYINGLGNYYKGKKNLAFFSYIAGGFGINIDSQIKSIVDETEICGSCINVHNMIELVKRNEKRAYSHEDLKKIFSVNREILLSDLC

SEQ ID NO: 243 - protein, 194 aa, synthetic construct
  REGION 1..194: note = Synthetic Construct
ITGADGKLVENTLLETYPNGAISGFMTEYFEMAFKGTEEAVNFEIATTELFKEVFGFETKHLGQTGSKSAPDVLLVSNNEGYQAIIDNKAYSKYSISGDHHNRMVHNYIENISKYSEYSHPIGFFTYIAGGFGNQIDRQIQSIVAECGVHGSGMTVSNMIKLVEKQNETPLSHRDIKNIFSVDRQIVLSDIEVI

SEQ ID NO: 244 - protein, 189 aa, synthetic construct
  REGION 1..189: note = Synthetic Construct
QTGFEDKLVEETLLKLYPRGSVGAFMTEYFEMAFKGRDEATDFEKATVELFQSVFGFQAKHVGPIGLTPDVLILSDAEGYQAILDNKAYSKYTISNDHHNRMVHNYIKNLKRYSNADVSLAFFSYIAGGFGNNINSQINDIVNVTGVAGSGISVSNMIKLVELYEPKNYTHKNIRDIFSVNRQILLSDL

SEQ ID NO: 245 - protein, 191 aa, synthetic construct
  REGION 1..191: note = Synthetic Construct
VTGVDGKLVENVLVETYPKGALGGFMTEYFEMAFKGTEEAIEFEKATTNLFQDVFGFNAIHLGQTGSKSAPDILLLSDSEGYQAIIDNKAYHKYSISGDHRNRMIHNYIESISNYSSFTQPIGFFSYVAGGFGNQIDKQIQDIADATGVHGSGITVSNMIELVKQQDIKPMNHAQIRTLFGVDRQIRIADF

SEQ ID NO: 246 - protein, 190 aa, synthetic construct
  REGION 1..190: note = Synthetic Construct
KSGVPFGNTEQILSKKYPYGFGDLFLQKYIELSRGGRKRATEFEKATSSIFADMFGVCAEHIGQKGSVPDIVVGSRDGKWAGILDTKAYNKKYSISNDHKNRMIGYIERYSEYGFEFANLSFFAYVVSDYGKNINSQIRYISNKSGVLGSAVTARDIIRMVERHQKKPYTHDEIREIFSVNRAITLKDID

SEQ ID NO: 247 - protein, 190 aa, synthetic construct
  REGION 1..190: note = Synthetic Construct
TTGIDERFVEETLLKFYPKGSIGAFMTEYFEMAFKGRDEATEFEKATVNIFQDVFGFSAKHVGPIGLTPDVLVLSDVDGYSAIIDNKAYSKYTINNDHHNRMVHNYIGNLSNYYDGTYSLAFFSYIAGGFGTNINKQLQSITNETGIKGSAMNVSNMIELIKRYDTCNYNHSTIREIFSVGRQILHSDFK

SEQ ID NO: 248 - protein, 189 aa, synthetic construct
  REGION 1..189: note = Synthetic Construct
KTGLAFSQVEELLLKLYPHGAVGAFMNEYFEMAFKGRDEATDFEKATVELFRDVFGFDAKHVGPIGLTPDVLLLSDSAGYCGIIDNKAYSKYTISNDHHNRMVHNYIGGFSNYCDSENELAFFSYIAGGFGSNIDKQLLKIIDETGVHGSAVTVSNIIKMVENQQKQPYSHIQIRDIFSLDRQIALSDI

SEQ ID NO: 249 - protein, 193 aa, synthetic construct
  REGION 1..193: note = Synthetic Construct
KSGINEKIVEEILLKFYPRGSVGAFMTEYFEMAFRGRDNATDFEKSTVQIFSDLFNYETIHVGSIGLTPDILILSDEDGYQAILDNKAYHSYSISNDHHNRMVHNYIAGLNKYSNSRLPLAFFSYISGGFGANINSQINKIYNETNIKGSAMTVSNMIYLIENYSEKSKSHRSLRKIFSVNRQILKSDIDIGL

SEQ ID NO: 250 - protein, 190 aa, synthetic construct
  REGION 1..190: note = Synthetic Construct
KSGVPFKDTERILSGKYPHGFKDRFLQEYIELSRSGRDKATEFEKATSSIFADVFGLRAEHIGQKGIVPDIVVASRGEKWAGILDTKSYKKKYSISNDHKNRMLEYIERYSEYGLEFANLSFFAYVVSDYGKNINSQLENISNRSGLLGSVITARYLARMVERHQKNPYSHEEIRKIFSVNRAITLKDID

SEQ ID NO: 251 - protein, 189 aa, synthetic construct
  REGION 1..189: note = Synthetic Construct
QTGFNDKLVEEVLLKLYPSGSIGGFMTAYFEMAFKGRDKATDFEKATVELFKNVFGFETKHVGPIGLTPDVLILSNSDGYQAIIDNKAYSKYTVSNDHRNRMIYNYIKNLKNYSNFSVPLSFFSYIAGGFGNNINSQIMDIVNATNIAGSAMSVSNMIKLVELYESKNYTHKNIKDIFSVNRQILLSDL

SEQ ID NO: 252 - protein, 189 aa, synthetic construct
  REGION 1..189: note = Synthetic Construct
QTGFGDKLVEETLLKLYPRGSIGAFMTEYFEMAFKGRDEAIDFEKATVELFQNVFGFESKHVGPIGLTPDVLILSDEDGYQAIIDNKAYSKYTISNDHHNRMVHNYIKNLERYSNSDVPLAFFSYVAGGFGKNINTQINDIVNVTGVSGSAMSVSNMIKLVELYESKNYTHKSIREIFSVNRQILLSDL

SEQ ID NO: 253 - protein, 189 aa, synthetic construct
  REGION 1..189: note = Synthetic Construct
KTGFEDKLIEETLLKLYPRGSVGAFMTEYFEMAFKGRDEASDFEKATVELFQNVFGFEAKHVGPIGLTPDVLILSDTDGYQAIIDNKAYSKYTISNDHHNRMVHNYIKDLNRYSSYTVPLAFFSYIAGGFGKNINSQVMDIVNVTKVSGSAISVSNMIKLVELYEQKNYTNKKIRDVFSVNRQILLSDL

SEQ ID NO: 254 - protein, 191 aa, synthetic construct
  REGION 1..191: note = Synthetic Construct
VTGVDGKLVENILVETYPKGALGGFMTEYFEMAFKGTEEAVEFEKATTNLFQDVFGFNAIHLGQTGSKSAPDILLLSDSEGYQAIIDNKAYSKYSITGDHKNRMIHNYIEHISNFSSFTQPIGFFSYVAGGFGNQIDKQIQDITSETGIHGSGITVSNMIELVKQQDIKPMNHAQIRTLFGVDRQIRMADF

SEQ ID NO: 255 - protein, 191 aa, synthetic construct
  REGION 1..191: note = Synthetic Construct
ITGTDRKLVEETLLSSYPHGLVGGFLANYYEMAFKGTEEAVEFEKATTEIFNSVFGYKAIHLGQTGSKSAPDILLLSDDEGYQAIIDNKAYSKYSITGDHHNRMVHNYIGKIGNYSESHYPLAFFSYIAGGFISTIDKQIASEVYESNVHGSGITVGTFIKMVEKHNATPYSHKELRNIFSVDREVKLADI

SEQ ID NO: 256 - protein, 190 aa, synthetic construct
  REGION 1..190: note = Synthetic Construct
ETGVSAVETERILSAKYPNGLVDSFLSEYVQMAFESRDRATEFEKATTSIFADIFGLYAEHIGQKGIVPDVVVASREEGWSGILDSKAYAKGYSIGHDHRNRMVEYIERYPKYGPEFATLAFFSYVVSDYKNSVTPQIRTISEKSGVPGSVITARDIVRMVERHQKKPYTHSEIREIFSLNRAITFEDIE

SEQ ID NO: 257 - protein, 189 aa, synthetic construct
  REGION 1..189: note = Synthetic Construct
QTGLDGKIVEETLLKLYPKGSVGAFMTEYFEMAFKGRDEATGFEKATVELFKNVFGYEAKHVGAIGLTPDVLILSDTDGYQAIIDNKAYSKYTISNDHHNRMVHNYIKGLNLYSTSSAPLAFFSYIAGGFGKNINSQIKGIVSETTIHGSAMSVSNMIRLVENYTDKGYKHSKIKEIFSLDRQILMSDI

SEQ ID NO: 258 - protein, 187 aa, synthetic construct
  REGION 1..187: note = Synthetic Construct
NEVTVEKYLQKNYPNGSIGAFMTSYFEMAFKGKDEAIDFEKATTEIFTSVFKYKAQHLGQTGSTSAPDILLISDEDGYQSIIDNKAYSEYSINGDHHNRMVHNYIRNIKNYSSCEYPIGYFSYIAGGFIKSIDKQIQAVASESGVNGSGITVGNFIKLIERNQIKPFSHKELRKIFGLNKQILLEDI

SEQ ID NO: 259 - protein, 194 aa, synthetic construct
  REGION 1..194: note = Synthetic Construct
RTGIDDRTVESYLIQNHRHGSLSEFFMAYRELAHSGRAGATDFELATCEIFQRLFHMRAKHVGPDGNTPDVFIESSECGYCGIIDNKAYHDKYSITAGHKRAMLVDYIPKYRGYGETDLPLAFYTYIAGSFGTNINNQLAAITKETGINGSAMPVDILIDFAQDYAERGCDHEYIKNLFSVNREIRLQDIATTK

SEQ ID NO: 260 - protein, 196 aa, synthetic construct; identical to SEQ ID NO: 1
  REGION 1..196: note = Synthetic Construct

SEQ ID NO: 261 - protein, 200 aa, synthetic construct; identical to SEQ ID NO: 2
  REGION 1..200: note = Synthetic Construct

SEQ ID NO: 262 - DNA, 21 bp, synthetic construct
  misc_feature 1..21: note = Synthetic Construct
  source 1..21: mol_type = other DNA
gacagccacctgctgggatct

SEQ ID NO: 263 - DNA, 128 bp, synthetic construct
  misc_feature 1..128: note = Synthetic Construct
  source 1..128: mol_type = other DNA
ggatcccctaagaaaaagcggaaggtgtgaaagcttctcgagtctagagggcccgtttaaacccgctgatcagcctcgactgtgccttctagttgccagccatctgttgtttgcccctcccccgtgcc

SEQ ID NO: 264 - DNA, 18 bp, synthetic construct
  misc_feature 1..18: note = Synthetic Construct
  source 1..18: mol_type = other DNA
acccccctcctcaccaca

SEQ ID NO: 265 - DNA, 18 bp, synthetic construct
  misc_feature 1..18: note = Synthetic Construct
  source 1..18: mol_type = other DNA
ataaggccagtagccagc

SEQ ID NO: 266 - DNA, 106 bp, synthetic construct
  misc_feature 1..106: note = Synthetic Construct
  source 1..106: mol_type = other DNA
ctggctaactagagaacccactgcttactggcttatcgaaattaatacgactcactatagggagtcccaagctggctagcgtttaaacttctgcggccgcgccacc

SEQ ID NO: 267 - DNA, 51 bp, synthetic construct
  misc_feature 1..51: note = Synthetic Construct
  source 1..51: mol_type = other DNA
atgggaaaacctattcctaatcctctgctgggcctggattctaccggaggc

SEQ ID NO: 268 - DNA, 408 bp, synthetic construct
  misc_feature 1..408: note = Synthetic Construct
  source 1..408: mol_type = other DNA
gtggacctgagaacactgggatattctcagcagcagcaggagaagatcaagcccaaggtgagatctacagtggcccagcaccacgaagccctggtgggacacggatttacacacgcccacattgtggccctgtctcagcaccctgccgccctgggaacagtggccgtgaaatatcaggatatgattgccgccctgcctgaggccacacacgaagccattgtgggagtgggaaaacgaggcgctggagccagagccctggaagccctgctgacagtggccggagaactgagaggacctcctctgcagctggatacaggacagctgctgaagattgccaaaaggggcggagtgaccgcggtggaagccgtgcacgcctggagaaatgccctgacaggagcccctctgaac

SEQ ID NO: 269 - DNA, 1794 bp, synthetic construct
  misc_feature 1..1794: note = Synthetic Construct
  source 1..1794: mol_type = other DNA
ctgacccccgaacaggtggtggccattgccagcaacatcggcggcaagcaggccctggaaaccgtgcagagactgctgcccgtgctgtgccaggcccatggcctgacacctgaacaggtggtggctatcgcctctcacgacggaggaaaacaggctctggaaacagtgcagcggctgctgcctgtgctgtgtcaggctcacggcttgactccagaacaggtggtggctattgcttcccacgacggggggaaacaggccctggaaactgtgcagcgcctgctgccagtgctgtgccaggctcacggactgacccccgaacaggtggtggccattgccagccacgacggcggcaagcaggccctggaaaccgtgcagagactgctgcccgtgctgtgccaggcccatggcctgacacctgaacaggtggtggctatcgcctctcacgacggaggaaaacaggctctggaaacagtgcagcggctgctgcctgtgctgtgtcaggctcacggcttgactccagaacaggtggtggctattgcttcccacgacggggggaaacaggccctggaaactgtgcagcgcctgctgccagtgctgtgccaggctcacgggctgacccccgaacaggtggtggccattgccagccacgacggcggcaagcaggccctggaaaccgtgcagagactgctgcccgtgctgtgccaggcccatggcctgacacctgaacaggtggtggctatcgcctctaacggcggaggaaaacaggctctggaaacagtgcagcggctgctgcctgtgctgtgtcaggctcacggcttgactccagaacaggtggtggctattgcttcccacgacggggggaaacaggccctggaaactgtgcagcgcctgctgccagtgctgtgccaggctcacggcctcactcccgaacaggtggtggccattgccagccacgacggcggcaagcaggccctggaaaccgtgcagagactgctgcccgtgctgtgccaggcccatggcctgacacctgaacaggtggtggctatcgcctctaacggcggaggaaaacaggctctggaaacagtgcagcggctgctgcctgtgctgtgtcaggctcacggcttgactccagaacaggtggtggctattgcttcccacgacggggggaaacaggccctggaaactgtgcagcgcctgctgccagtgctgtgccaggctcacggactgacccccgaacaggtggtggccattgccagcaacatcggcggcaagcaggccctggaaaccgtgcagagactgctgcccgtgctgtgccaggcccatggcctgacacctgaacaggtggtggctatcgcctctcacgacggaggaaaacaagcactcgagacagtgcagcggctgctgcctgtgctgtgtcaggctcacggcttgactccagaacaggtggtggctattgcttcccacgacggggggaaacaggccctggaaactgtgcagcgcctgctgccagtgctgtgccaggctcacggcctgacccccgaacaggtggtggccattgccagcaacatcggcggcaagcaggccctggaaaccgtgcagagactgctgcccgtgctgtgccaggcccatggcctgacacctgaacaggtggtggctatcgcctctcacgacggaggaaaacaggctctggaaacagtgcagcggctgctgcctgtgctgtgtcaggctcacggcttgactccacagcaggtcgtggcaattgctagcaatatcggcggacggcccgccctggag

SEQ ID NO: 270 - DNA, 150 bp, synthetic construct
  misc_feature 1..150: note = Synthetic Construct
  source 1..150: mol_type = other DNA
agcattgtggcccagctgtctagacctgatcctgccctggccgccctgacaaatgatcacctggtggccctggcctgtctgggaggcagacctgccctggatgccgtgaaaaaaggactgcctcacgcccctgccctgatcaagagaaca

SEQ ID NO: 271 - DNA, 29 bp, synthetic construct
  misc_feature 1..29: note = Synthetic Construct
  source 1..29: mol_type = other DNA
ggatcccctaagaaaaagcggaaggtggg

SEQ ID NO: 272 - DNA, 21 bp, synthetic construct
  misc_feature 1..21: note = Synthetic Construct
  source 1..21: mol_type = other DNA
atctgtgagcaggtgcaggag

SEQ ID NO: 273 - DNA, 106 bp, synthetic construct; identical to SEQ ID NO: 266
  misc_feature 1..106: note = Synthetic Construct
  source 1..106: mol_type = other DNA

SEQ ID NO: 274 - DNA, 51 bp, synthetic construct; identical to SEQ ID NO: 267
  misc_feature 1..51: note = Synthetic Construct
  source 1..51: mol_type = other DNA

SEQ ID NO: 275 - DNA, 408 bp, synthetic construct; identical to SEQ ID NO: 268
  misc_feature 1..408: note = Synthetic Construct
  source 1..408: mol_type = other DNA

SEQ ID NO: 276 - DNA, 1794 bp, synthetic construct
  misc_feature 1..1794: note = Synthetic Construct
  source 1..1794: mol_type = other DNA
ctgacccccgaacaggtggtggccattgccagcaacatcggcggcaagcaggccctggaaaccgtgcagagactgctgcccgtgctgtgccaggcccatggcctgacacctgaacaggtggtggctatcgcctctaacggcggaggaaaacaggctctggaaacagtgcagcggctgctgcctgtgctgtgtcaggctcacggcttgactccagaacaggtggtggctattgcttccaatattggggggaaacaggccctggaaactgtgcagcgcctgctgccagtgctgtgccaggctcacggactgacccccgaacaggtggtggccattgccagcaacatcggcggcaagcaggccctggaaaccgtgcagagactgctgcccgtgctgtgccaggcccatggcctgacacctgaacaggtggtggctatcgcctctaacaacggaggaaaacaggctctggaaacagtgcagcggctgctgcctgtgctgtgtcaggctcacggcttgactccagaacaggtggtggctattgcttccaacaacggggggaaacaggccctggaaactgtgcagcgcctgctgccagtgctgtgccaggctcacgggctgacccccgaacaggtggtggccattgccagccacgacggcggcaagcaggccctggaaaccgtgcagagactgctgcccgtgctgtgccaggcccatggcctgacacctgaacaggtggtggctatcgcctctcacgacggaggaaaacaggctctggaaacagtgcagcggctgctgcctgtgctgtgtcaggctcacggcttgactccagaacaggtggtggctattgcttccaatattggggggaaacaggccctggaaactgtgcagcgcctgctgccagtgctgtgccaggctcacggcctcactcccgaacaggtggtggccattgccagcaacaacggcggcaagcaggccctggaaaccgtgcagagactgctgcccgtgctgtgccaggcccatggcctgacacctgaacaggtggtggctatcgcctctaacggcggaggaaaacaggctctggaaacagtgcagcggctgctgcctgtgctgtgtcaggctcacggcttgactccagaacaggtggtggctattgcttccaatattggggggaaacaggccctggaaactgtgcagcgcctgctgccagtgctgtgccaggctcacggactgacccccgaacaggtggtggccattgccagcaacaacggcggcaagcaggccctggaaaccgtgcagagactgctgcccgtgctgtgccaggcccatggcctgacacctgaacaggtggtggctatcgcctctcacgacggaggaaaacaagcactcgagacagtgcagcggctgctgcctgtgctgtgtcaggctcacggcttgactccagaacaggtggtggctattgcttcccacgacggggggaaacaggccctggaaactgtgcagcgcctgctgccagtgctgtgccaggctcacggcctgacccccgaacaggtggtggccattgccagcaacatcggcggcaagcaggccctggaaaccgtgcagagactgctgcccgtgctgtgccaggcccatggcctgacacctgaacaggtggtggctatcgcctctaacaacggaggaaaacaggctctggaaacagtgcagcggctgctgcctgtgctgtgtcaggctcacggcttgactccacagcaggtcgtggcaattgctagccacgacggcggacggcccgccctggag

SEQ ID NO: 277 - DNA, 150 bp, synthetic construct; identical to SEQ ID NO: 270
  misc_feature 1..150: note = Synthetic Construct
  source 1..150: mol_type = other DNA

SEQ ID NO: 278 - DNA, 29 bp, synthetic construct
  misc_feature 1..29: note = Synthetic Construct
  source 1..29: mol_type = other DNA
ggatcccctaagaaaaagcggaaggtggg

SEQ ID NO: 279 - DNA, 21 bp, synthetic construct
  misc_feature 1..21: note = Synthetic Construct
  source 1..21: mol_type = other DNA
atctgtgagcaggtgcaggag

SEQ ID NO: 280 - DNA, 18 bp, synthetic construct
  misc_feature 1..18: note = Synthetic Construct
  source 1..18: mol_type = other DNA
acccccctcctcaccaca

SEQ ID NO: 281 - DNA, 18 bp, synthetic construct
  misc_feature 1..18: note = Synthetic Construct
  source 1..18: mol_type = other DNA
ataaggccagtagccagc

SEQ ID NO: 282 - protein, 186 aa, synthetic construct
  REGION 1..186: note = Synthetic Construct
TGIPSKYIEEQLDSFRIDTFSLFETNYIDMAFSGREFASEFEHTTMDVFSELGFQTQHVGTKSRQPDIFIQSHDASFSGIIDNKAYHVFSITHDYELKMINSYIPKYKKRYSDFSFFMYIAGGFGKNFDKQVQTIANQSGINGCGIRASDLMRLLKKHKQNPIDHQKLKQIFECNRLVRIQDILSL

SEQ ID NO: 283 - DNA, 701 bp, synthetic construct
  misc_feature 1..701: note = Synthetic Construct
  source 1..701: mol_type = other DNA
gacagccacctgctgggatctatccccagcaagtacatcgaggaacagctggacagcttccggatcgacaccttcagcctgttcgagacaaactacatcgacatggccttcagcggcagagagttcgccagcgagtttgagcacaccaccatggacgtgttcagcgagctgggctttcagacacagcacgtgggcaccaagagcagacagcccgacatcttcatccagagccacgacgccagcttctccggcatcatcgacaacaaggcctaccacgtgttctctatcacccacgactacgagctgaagatgatcaacagctacatccccaagtacaagaagcggtacagcgacttcagcttcttcatgtacattgccggcggattcggcaagaacttcgacaaacaggtgcagacaatcgccaaccagagcggcatcaatggctgcggcattagagccagcgacctgatgagactgctgaagaagcacaagcagaaccccatcgaccaccagaaactgaagcagatcttcgagtgcaaccggctcgtgcggatccaggatattctgagccttggatcccctaagaaaaagcggaaggtgtgaaagcttctcgagtctagagggcccgtttaaacccgctgatcagcctcgactgtgccttctagttgccagccatctgttgtttgcccctcccccgtgcc

SEQ ID NO: 284 - DNA, 106 bp, synthetic construct; identical to SEQ ID NO: 266
  misc_feature 1..106: note = Synthetic Construct
  source 1..106: mol_type = other DNA

SEQ ID NO: 285 - DNA, 51 bp, synthetic construct; identical to SEQ ID NO: 267
  misc_feature 1..51: note = Synthetic Construct
  source 1..51: mol_type = other DNA

SEQ ID NO: 286 - DNA, 408 bp, synthetic construct; identical to SEQ ID NO: 268
  misc_feature 1..408: note = Synthetic Construct
  source 1..408: mol_type = other DNA

SEQ ID NO: 287 - DNA, 1794 bp, synthetic construct
  misc_feature 1..1794: note = Synthetic Construct
  source 1..1794: mol_type = other DNA
ctgacccccgaacaggtggtggccattgccagcaacaacggcggcaagcaggccctggaaaccgtgcagagactgctgcccgtgctgtgccaggcccatggcctgacacctgaacaggtggtggctatcgcctctaatatcggaggaaaacaggctctggaaacagtgcagcggctgctgcctgtgctgtgtcaggctcacggcttgactccagaacaggtggtggctattgcttccaacggcggggggaaacaggccctggaaactgtgcagcgcctgctgccagtgctgtgccaggctcacggactgacccccgaacaggtggtggccattgccagccacgacggcggcaagcaggccctggaaaccgtgcagagactgctgcccgtgctgtgccaggcccatggcctgacacctgaacaggtggtggctatcgcctctcacgacggaggaaaacaggctctggaaacagtgcagcggctgctgcctgtgctgtgtcaggctcacggcttgactccagaacaggtggtggctattgcttccaacggcggggggaaacaggccctggaaactgtgcagcgcctgctgccagtgctgtgccaggctcacgggctgacccccgaacaggtggtggccattgccagccacgacggcggcaagcaggccctggaaaccgtgcagagactgctgcccgtgctgtgccaggcccatggcctgacacctgaacaggtggtggctatcgcctctaacggcggaggaaaacaggctctggaaacagtgcagcggctgctgcctgtgctgtgtcaggctcacggcttgactccagaacaggtggtggctattgcttccaacggcggggggaaacaggccctggaaactgtgcagcgcctgctgccagtgctgtgccaggctcacggcctcactcccgaacaggtggtggccattgccagcaacaacggcggcaagcaggccctggaaaccgtgcagagactgctgcccgtgctgtgccaggcccatggcctgacacctgaacaggtggtggctatcgcctctaacggcggaggaaaacaggctctggaaacagtgcagcggctgctgcctgtgctgtgtcaggctcacggcttgactccagaacaggtggtggctattgcttcccacgacggggggaaacaggccctggaaactgtgcagcgcctgctgccagtgctgtgccaggctcacggactgacccccgaacaggtggtggccattgccagccacgacggcggcaagcaggccctggaaaccgtgcagagactgctgcccgtgctgtgccaggcccatggcctgacacctgaacaggtggtggctatcgcctctcacgacggaggaaaacaagcactcgagacagtgcagcggctgctgcctgtgctgtgtcaggctcacggcttgactccagaacaggtggtggctattgcttccaatattggggggaaacaggccctggaaactgtgcagcgcctgctgccagtgctgtgccaggctcacggcctgacccccgaacaggtggtggccattgccagccacgacggcggcaagcaggccctggaaaccgtgcagagactgctgcccgtgctgtgccaggcccatggcctgacacctgaacaggtggtggctatcgcctctaatatcggaggaaaacaggctctggaaacagtgcagcggctgctgcctgtgctgtgtcaggctcacggcttgactccacagcaggtcgtggcaattgctagcaacaacggcggacggcccgccctggag

SEQ ID NO: 288 - DNA, 17 bp, synthetic construct
  misc_feature 1..17: note = Synthetic Construct
  source 1..17: mol_type = other DNA
agcatgagaccccggaa

SEQ ID NO: 289 - DNA, 106 bp, synthetic construct; identical to SEQ ID NO: 266
  misc_feature 1..106: note = Synthetic Construct
  source 1..106: mol_type = other DNA

SEQ ID NO: 290 - DNA, 50 bp, synthetic construct
  misc_feature 1..50: note = Synthetic Construct
  source 1..50: mol_type = other DNA
atgggaaaacctattcctaatcctctgctgggcctggattctaccggagg

SEQ ID NO: 291 - DNA, 408 bp, synthetic construct; identical to SEQ ID NO: 268
  misc_feature 1..408: note = Synthetic Construct
  source 1..408: mol_type = other DNA

SEQ ID NO: 292 - DNA, 1794 bp, synthetic construct
  misc_feature 1..1794: note = Synthetic Construct
  source 1..1794: mol_type = other DNA
ctgacccccgaacaggtggtggccattgccagcaacatcggcggcaagcaggccctggaaaccgtgcagagactgctgcccgtgctgtgccaggcccatggcctgacacctgaacaggtggtggctatcgcctctaacaacggaggaaaacaggctctggaaacagtgcagcggctgctgcctgtgctgtgtcaggctcacggcttgactccagaacaggtggtggctattgcttcccacgacggggggaaacaggccctggaaactgtgcagcgcctgctgccagtgctgtgccaggctcacggactgacccccgaacaggtggtggccattgccagcaacggcggcggcaagcaggccctggaaaccgtgcagagactgctgcccgtgctgtgccaggcccatggcctgacacctgaacaggtggtggctatcgcctctaacaacggaggaaaacaggctctggaaacagtgcagcggctgctgcctgtgctgtgtcaggctcacggcttgactccagaacaggtggtggctattgcttccaacaacggggggaaacaggccctggaaactgtgcagcgcctgctgccagtgctgtgccaggctcacgggctgacccccgaacaggtggtggccattgccagcaacggcggcggcaagcaggccctggaaaccgtgcagagactgctgcccgtgctgtgccaggcccatggcctgacacctgaacaggtggtggctatcgcctctaatatcggaggaaaacaggctctggaaacagtgcagcggctgctgcctgtgctgtgtcaggctcacggcttgactccagaacaggtggtggctattgcttcccacgacggggggaaacaggccctggaaactgtgcagcgcctgctgccagtgctgtgccaggctcacggcctcactcccgaacaggtggtggccattgccagcaacatcggcggcaagcaggccctggaaaccgtgcagagactgctgcccgtgctgtgccaggcccatggcctgacacctgaacaggtggtggctatcgcctctcacgacggaggaaaacaggctctggaaacagtgcagcggctgctgcctgtgctgtgtcaggctcacggcttgactccagaacaggtggtggctattgcttccaacaacggggggaaacaggccctggaaactgtgcagcgcctgctgccagtgctgtgccaggctcacggactgacccccgaacaggtggtggccattgccagcaacaacggcggcaagcaggccctggaaaccgtgcagagactgctgcccgtgctgtgccaggcccatggcctgacacctgaacaggtggtggctatcgcctctcacgacggaggaaaacaagcactcgagacagtgcagcggctgctgcctgtgctgtgtcaggctcacggcttgactccagaacaggtggtggctattgcttccaatattggggggaaacaggccctggaaactgtgcagcgcctgctgccagtgctgtgccaggctcacggcctgacccccgaacaggtggtggccattgccagcaacaacggcggcaagcaggccctggaaaccgtgcagagactgctgcccgtgctgtgccaggcccatggcctgacacctgaacaggtggtggctatcgcctctaacaacggaggaaaacaggctctggaaacagtgcagcggctgctgcctgtgctgtgtcaggctcacggcttgactccacagcaggtcgtggcaattgctagcaacaacggcggacggcccgccctggag

SEQ ID NO: 293 - DNA, 17 bp, synthetic construct
  misc_feature 1..17: note = Synthetic Construct
  source 1..17: mol_type = other DNA
agcatgagaccccggaa

SEQ ID NO: 294 - DNA, 18 bp, synthetic construct
  misc_feature 1..18: note = Synthetic Construct
  source 1..18: mol_type = other DNA
gatcctcttgtcccacag

SEQ ID NO: 295 - DNA, 18 bp, synthetic construct
  misc_feature 1..18: note = Synthetic Construct
  source 1..18: mol_type = other DNA
agctggtacacggcaggg

SEQ ID NO: 296 - protein, 185 aa, synthetic construct
  REGION 1..185: note = Synthetic Construct
GIPSKYIEEQLDSFRIDTFSLFETNYIDMAFSGREFASEFEHTTMDVFSELGFQTQHVGTKSRQPDIFIQSHDASFSGIIDNKAYHVFSITHDYELKMINSYIPKYKKRYSDFSFFMYIAGGFGKNFDKQVQTIANQSGINGCGIRASDLMRLLKKHKQNPIDHQKLKQIFECNRLVRIQDILSL

SEQ ID NO: 297 - protein, 187 aa, synthetic construct
  REGION 1..187: note = Synthetic Construct
KTGIPSKYIEEQLDSFRIDTFSLFETNYIDMAFSGREFASEFEHTTMDVFSELGFQTQHVGTKSRQPDIFIQSHDASFSGIIDNKAYHVFSITHDYELKMINSYIPKYKKRYSDFSFFMYIAGGFGKNFDKQVQTIANQSGINGCGIRASDLMRLLKKHKQNPIDHQKLKQIFECNRLVRIQDILSL

SEQ ID NO: 298 - protein, 188 aa, synthetic construct
  REGION 1..188: note = Synthetic Construct
SKTGIPSKYIEEQLDSFRIDTFSLFETNYIDMAFSGREFASEFEHTTMDVFSELGFQTQHVGTKSRQPDIFIQSHDASFSGIIDNKAYHVFSITHDYELKMINSYIPKYKKRYSDFSFFMYIAGGFGKNFDKQVQTIANQSGINGCGIRASDLMRLLKKHKQNPIDHQKLKQIFECNRLVRIQDILSL

SEQ ID NO: 299 - protein, 189 aa, synthetic construct
  REGION 1..189: note = Synthetic Construct
ASKTGIPSKYIEEQLDSFRIDTFSLFETNYIDMAFSGREFASEFEHTTMDVFSELGFQTQHVGTKSRQPDIFIQSHDASFSGIIDNKAYHVFSITHDYELKMINSYIPKYKKRYSDFSFFMYIAGGFGKNFDKQVQTIANQSGINGCGIRASDLMRLLKKHKQNPIDHQKLKQIFECNRLVRIQDILSL